European Patent Specification EP 3 668 898 B1, published July 5, 2023. Title: HUMANIZED ANTIBODIES FOR CD3. Applicant: MORPHOSYS AG. Application EP 17186128.9. The sequence listing filed with the application follows.

SEQUENCE LISTING (157 sequences)

SEQ ID NO: 1 - protein, 104 aa, Homo sapiens
DGNEEMGGITQTPYKVSISGTTVILTCPQYPGSEILWQHNDKNIGGDEDDKNIGSDEDHLSLKEFSELEQSGYYVCYPRGSKPEDANFYLYLRARVCENCMEMD

SEQ ID NO: 2 - protein, 96 aa, Macaca fascicularis
QDGNEEMGSITQTPYQVSISGTTVILTCSQHLGSEAQWQHNGKNKEDSGDRLFLPEFSEMEQSGYYVCYPRGSNPEDASHHLYLKARVCENCMEMD

SEQ ID NO: 3 - protein, 125 aa, Artificial Sequence
  source: /note="Description of Artificial Sequence: Synthetic polypeptide"
EVQLVESGGGLVQPKGSLKLSCAASGFTFNTYAMNWVRQAPGKGLEWVARIRSKYNNYATYYADSVKDRFTISRDDSQSILYLQMNNLKTEDTAMYYCVRHGNFGNSYVSWFAYWGQGTLVTVSS

SEQ ID NO: 4 - protein, 111 aa, Artificial Sequence
  source: /note="Description of Artificial Sequence: Synthetic polypeptide"
QAVVTQESALTTSPGETVTLTCRSSTGAVTTSNYANWVQEKPDHLFTGLIGGTNKRAPGVPARFSGSLIGDKAALTITGAQTEDEAIYFCALWYSNLWVFGGGTKLTVLGQ

SEQ ID NO: 5 - protein, 125 aa, Artificial Sequence
  source: /note="Description of Artificial Sequence: Synthetic polypeptide"
EVQLVESGGGLVQPGGSLKLSCAASGFTFNKYAMNWVRQAPGKGLEWVARIRSKYNNYATYYADSVKDRFTISRDDSKNTAYLQMNNLKTEDTAVYYCVRHGNFGNSYISYWAYWGQGTLVTVSS

SEQ ID NO: 6 - protein, 111 aa, Artificial Sequence
  source: /note="Description of Artificial Sequence: Synthetic polypeptide"
QTVVTQEPSLTVSPGGTVTLTCGSSTGAVTSGNYPNWVQQKPGQAPRGLIGGTKFLAPGTPARFSGSLLGGKAALTLSGVQPEDEAEYYCVLWYSNRWVFGGGTKLTVLGQ

SEQ ID NO: 7 - protein, 125 aa, Artificial Sequence
  source: /note="Description of Artificial Sequence: Synthetic polypeptide"
EVQLVESGGGLVKPGGSLRLSCAASGFTFNTYAMNWVRQAPGKGLEWVGRIRSKYNNYATYYADSVKDRFTISRDDSKNTLYLQMNSLKTEDTAVYYCTTHGNFGNSYVSWFAYWGQGTLVTVSS

SEQ ID NO: 8 - DNA, 375 bp, Artificial Sequence
  source: /note="Description of Artificial Sequence: Synthetic polynucleotide"
gaagtgcagctggtggaatctggcggcggactcgtgaagcctggcggctctctgagactgagctgtgccgccagcggcttcaccttcaacacctacgccatgaactgggtgcgccaggcccctggcaaaggcctggaatgggtgggacggatcagaagcaagtacaacaattacgccacctactacgccgacagcgtgaaggaccggttcaccatcagccgggacgacagcaagaacaccctgtacctgcagatgaacagcctgaaaaccgaggacaccgccgtgtactactgcaccacccacggcaacttcggcaacagctatgtgtcttggtttgcctactggggccagggcaccctcgtgacagtctcgagc

SEQ ID NO: 9 - protein, 125 aa, Artificial Sequence
  source: /note="Description of Artificial Sequence: Synthetic polypeptide"
QVQLVESGGGLVKPGGSLRLSCAASGFTFNTYAMNWIRQAPGKGLEWVSRIRSKYNNYATYYADSVKDRFTISRDNAKNSLYLQMNSLRAEDTAVYYCVRHGNFGNSYVSWFAYWGQGTLVTVSS

SEQ ID NO: 10 - DNA, 375 bp, Artificial Sequence
  source: /note="Description of Artificial Sequence: Synthetic polynucleotide"
caggtgcagctggtggaatctggcggcggactcgtgaagcctggcggctctctgagactgagctgtgccgccagcggcttcaccttcaacacctacgccatgaactggatccggcaggcccctggcaagggcctggaatgggtgtcccggatcagaagcaagtacaacaattacgccacctactacgccgacagcgtgaaggaccggttcaccatcagccgggacaacgccaagaacagcctgtacctgcagatgaactccctgcgggccgaggacaccgccgtgtactattgtgtgcggcacggcaacttcggcaacagctatgtgtcttggtttgcctactggggccagggcaccctcgtgacagtctcgagc

SEQ ID NO: 11 - protein, 111 aa, Artificial Sequence
  source: /note="Description of Artificial Sequence: Synthetic polypeptide"
QAVVTQEPSLTVSPGGTVTLTCRSSTGAVTTSNYANWVQQKPGQAPRGLIGGTNKRAPWTPARFSGSLLGGKAALTITGAQAEDEADYYCALWYSNLWVFGGGTKLTVLGQ

SEQ ID NO: 12 - DNA, 333 bp, Artificial Sequence
  source: /note="Description of Artificial Sequence: Synthetic polynucleotide"
caggccgtggttacacaagagcccagcctgacagttagccctggcggaacagtgaccctgacctgcagatcttctacaggcgccgtgaccaccagcaactacgccaattgggtgcagcagaagcctggacaggctcccagaggactgatcggcggcacaaacaaaagagccccttggacacccgccagattcagcggatcactgctcggaggaaaggccgcactgacaatcacaggtgcccaggccgaagatgaggccgattactattgcgccctgtggtacagcaacctgtgggtgttcggcggaggtaccaagctgaccgtgctgggccag

SEQ ID NO: 13 - protein, 111 aa, Artificial Sequence
  source: /note="Description of Artificial Sequence: Synthetic polypeptide"
ELVVTQEPSLTVSPGGTVTLTCRSSTGAVTTSNYANWVQQKPGQAPRGLIGGTNKRAPGTPARFSGSLLGGKAALTLSGVQPEDEAEYYCALWYSNLWVFGGGTKLTVLGQ

SEQ ID NO: 14 - DNA, 333 bp, Artificial Sequence
  source: /note="Description of Artificial Sequence: Synthetic polynucleotide"
gagctggtggtcacacaagagcccagcctgacagtttctcctggcggcacagtgaccctgacctgcagatcttctacaggcgccgtgaccacctccaactacgccaattgggtgcagcagaagcctggacaggctcccagaggactgatcggcggcacaaacaaaagagcccctggcacaccagccagattcagcggatcactgctcggaggaaaggccgctctgacactgtctggtgtccagcctgaagatgaggccgagtactactgcgccctgtggtacagcaatctgtgggtgttcggcggaggtaccaagctgaccgtgctgggccag

SEQ ID NO: 15 - protein, 111 aa, Artificial Sequence
  source: /note="Description of Artificial Sequence: Synthetic polypeptide"
QTVVTQEPSLTVSPGGTVTLTCRSSTGAVTTSNYANWVQQKPGQAPRGLIGGTNKRAPGTPARFSGSLLGGKAALTLLGAQPEDEAEYYCALWYSNLWVFGGGTKLTVLGQ

SEQ ID NO: 16 - DNA, 333 bp, Artificial Sequence
  source: /note="Description of Artificial Sequence: Synthetic polynucleotide"
cagaccgtggtcacacaagagcccagcctgacagtttctcctggcggcacagtgaccctgacctgcagatcttctacaggcgccgtgaccaccagcaactacgccaattgggtgcagcagaagcctggacaggctcccagaggactgatcggcggcacaaacaaaagagcccctggcacaccagccagattcagcggatcactgctcggaggaaaggccgctctgacactgcttggagcacagcctgaagatgaggccgagtactactgcgccctgtggtacagcaatctgtgggtgttcggcggaggtaccaagctgaccgtgctgggccag

SEQ ID NO: 17 - protein, 111 aa, Artificial Sequence
  source: /note="Description of Artificial Sequence: Synthetic polypeptide"
QTVVTQEPSLTVSPGGTVTLTCRSSTGAVTTSNYANWVQQKPGQAPRGLIGGTKFLAPGTPARFSGSLLGGKAALTLLGAQPEDEAEYYCALWYSNLWVFGGGTKLTVLGQ

SEQ ID NO: 18 - DNA, 333 bp, Artificial Sequence
  source: /note="Description of Artificial Sequence: Synthetic polynucleotide"
cagaccgtggtcacacaagagcccagcctgacagtttctcctggcggcacagtgaccctgacctgcagatcttctacaggcgccgtgaccaccagcaactacgccaattgggtgcagcagaagcctggacaggctcccagaggactgatcggcggcacaaaatttctggcccctggcacaccagccagattctctggatctctgctcggcggaaaggccgctctgacactgcttggagcacagcctgaagatgaggccgagtactactgcgccctgtggtacagcaatctgtgggtgttcggcggaggtaccaagctgaccgtgctgggccag

SEQ ID NO: 19 - protein, 111 aa, Artificial Sequence
  source: /note="Description of Artificial Sequence: Synthetic polypeptide"
QTVVTQEPSLTVSPGGTVTLTCRSSTGAVTTSNYANWVQQKPGQAPRGLIGGTKFLAPGTPARFSGSLLGGKAALTLSGVQPEDEAEYYCALWYSNLWVFGGGTKLTVLGQ

SEQ ID NO: 20 - DNA, 333 bp, Artificial Sequence
  source: /note="Description of Artificial Sequence: Synthetic polynucleotide"
cagaccgtggtcacacaagagcccagcctgacagtttctcctggcggcacagtgaccctgacctgcagatcttctacaggcgccgtgaccaccagcaactacgccaattgggtgcagcagaagcctggacaggctcccagaggactgatcggcggcacaaaatttctggcccctggcacaccagccagattctctggatctctgctcggcggaaaggccgctctgacactgtctggtgttcagcctgaggacgaggccgagtactattgcgccctgtggtacagcaacctgtgggtgttcggcggaggtaccaagctgaccgtgctgggccag

SEQ ID NO: 21 - protein, 111 aa, Artificial Sequence
  source: /note="Description of Artificial Sequence: Synthetic polypeptide"
QTVVTQEPSLTVSPGGTVTLTCRSSTGAVTTSNYANWVQQKPGQAPRGLIGGTNKRAPGTPARFSGSLLGGKAALTLSGVQPEDEAEYYCALWYSNLWVFGGGTKLTVLGQ

SEQ ID NO: 22 - DNA, 333 bp, Artificial Sequence
  source: /note="Description of Artificial Sequence: Synthetic polynucleotide"
cagaccgtggtcacacaagagcccagcctgacagtttctcctggcggcacagtgaccctgacctgcagatcttctacaggcgccgtgaccaccagcaactacgccaattgggtgcagcagaagcctggacaggctcccagaggactgatcggcggcacaaacaaaagagcccctggcacaccagccagattcagcggatcactgctcggaggaaaggccgctctgacactgtctggtgtccagcctgaagatgaggccgagtactactgcgccctgtggtacagcaatctgtgggtgttcggcggaggtaccaagctgaccgtgctgggccag

SEQ ID NO: 23 - protein, 5 aa, Artificial Sequence
  source: /note="Description of Artificial Sequence: Synthetic peptide"
TYAMN

SEQ ID NO: 24 - protein, 19 aa, Artificial Sequence
  source: /note="Description of Artificial Sequence: Synthetic peptide"
RIRSKYNNYATYYADSVKD

SEQ ID NO: 25 - protein, 14 aa, Artificial Sequence
  source: /note="Description of Artificial Sequence: Synthetic peptide"
HGNFGNSYVSWFAY

SEQ ID NO: 26 - protein, 14 aa, Artificial Sequence
  source: /note="Description of Artificial Sequence: Synthetic peptide"
RSSTGAVTTSNYAN

SEQ ID NO: 27 - protein, 7 aa, Artificial Sequence
  source: /note="Description of Artificial Sequence: Synthetic peptide"
GTNKRAP

SEQ ID NO: 28 - protein, 9 aa, Artificial Sequence
  source: /note="Description of Artificial Sequence: Synthetic peptide"
ALWYSNLWV

SEQ ID NO: 29 - protein, 111 aa, Artificial Sequence; identical to SEQ ID NO: 11
  source: /note="Description of Artificial Sequence: Synthetic polypeptide"

SEQ ID NO: 30 - protein, 125 aa, Artificial Sequence; identical to SEQ ID NO: 9
  source: /note="Description of Artificial Sequence: Synthetic polypeptide"

SEQ ID NO: 31 - DNA, 333 bp, Artificial Sequence; identical to SEQ ID NO: 12
  source: /note="Description of Artificial Sequence: Synthetic polynucleotide"

SEQ ID NO: 32 - DNA, 375 bp, Artificial Sequence; identical to SEQ ID NO: 10
  source: /note="Description of Artificial Sequence: Synthetic polynucleotide"

SEQ ID NO: 33 - DNA, 12 bp, Artificial Sequence
  source: /note="Description of Artificial Sequence: Synthetic oligonucleotide"
acctacgccatg

SEQ ID NO: 34 - DNA, 57 bp, Artificial Sequence
  source: /note="Description of Artificial Sequence: Synthetic oligonucleotide"
cggatcagaagcaagtacaacaattacgccacctactacgccgacagcgtgaaggac

SEQ ID NO: 35 - DNA, 42 bp, Artificial Sequence
  source: /note="Description of Artificial Sequence: Synthetic oligonucleotide"
cacggcaacttcggcaacagctatgtgtcttggtttgcctac

SEQ ID NO: 36 - DNA, 42 bp, Artificial Sequence
  source: /note="Description of Artificial Sequence: Synthetic oligonucleotide"
agatcttctacaggcgccgtgaccaccagcaactacgccaat

SEQ ID NO: 37 - DNA, 21 bp, Artificial Sequence
  source: /note="Description of Artificial Sequence: Synthetic oligonucleotide"
ggcacaaacaaaagagcccct

SEQ ID NO: 38 - DNA, 27 bp, Artificial Sequence
  source: /note="Description of Artificial Sequence: Synthetic oligonucleotide"
gccctgtggtacagcaatctgtgggtg

SEQ ID NO: 39 - protein, 215 aa, Artificial Sequence
  source: /note="Description of Artificial Sequence: Synthetic polypeptide"
QAVVTQEPSLTVSPGGTVTLTCRSSTGAVTTSNYANWVQQKPGQAPRGLIGGTNKRAPWTPARFSGSLLGGKAALTITGAQAEDEADYYCALWYSNLWVFGGGTKLTVLGQPKAAPSVTLFPPSSEELQANKATLVCLISDFYPGAVTVAWKADSSPVKAGVETTTPSKQSNNKYAASSYLSLTPEQWKSHRSYSCQVTHEGSTVEKTVAPTECS

SEQ ID NO: 40 - protein, 455 aa, Artificial Sequence
  source: /note="Description of Artificial Sequence: Synthetic polypeptide"
QVQLVESGGGLVKPGGSLRLSCAASGFTFNTYAMNWIRQAPGKGLEWVSRIRSKYNNYATYYADSVKDRFTISRDNAKNSLYLQMNSLRAEDTAVYYCVRHGNFGNSYVSWFAYWGQGTLVTVSSASTKGPSVFPLAPSSKSTSGGTAALGCLVKDYFPEPVTVSWNSGALTSGVHTFPAVLQSSGLYSLSSVVTVPSSSLGTQTYICNVNHKPSNTKVDKRVEPKSCDKTHTCPPCPAPELLGGPSVFLFPPKPKDTLMISRTPEVTCVVVDVSHEDPEVKFNWYVDGVEVHNAKTKPREEQYNSTYRVVSVLTVLHQDWLNGKEYKCKVSNKALPAPIEKTISKAKGQPREPQVYTLPPSREEMTKNQVSLTCLVKGFYPSDIAVEWESNGQPENNYKTTPPVLDSDGSFFLYSKLTVDKSRWQQGNVFSCSVMHEALHNHYTQKSLSLSPGK

SEQ ID NO: 41 - DNA, 645 bp, Artificial Sequence
  source: /note="Description of Artificial Sequence: Synthetic polynucleotide"
caggccgtggttacacaagagcccagcctgacagttagccctggcggaacagtgaccctgacctgcagatcttctacaggcgccgtgaccaccagcaactacgccaattgggtgcagcagaagcctggacaggctcccagaggactgatcggcggcacaaacaaaagagccccttggacacccgccagattcagcggatcactgctcggaggaaaggccgcactgacaatcacaggtgcccaggccgaagatgaggccgattactattgcgccctgtggtacagcaacctgtgggtgttcggcggaggtaccaagctgaccgtgctgggccagcccaaagccgcccctagcgtgaccctgttccccccctcgagtgaggaactccaggccaacaaggccaccctcgtgtgcctgatcagcgacttctaccctggcgccgtgaccgtggcctggaaggccgatagcagccctgtgaaggccggcgtggaaaccaccacccccagcaagcagagcaacaacaaatacgccgccagcagctacctgagcctgacccccgagcagtggaagtcccacagatcctacagctgccaggtcacacacgagggcagcaccgtggaaaagaccgtggcccccaccgagtgcagc

SEQ ID NO: 42 - DNA, 1368 bp, Artificial Sequence
  source: /note="Description of Artificial Sequence: Synthetic polynucleotide"
caggtgcagctggtggaatctggcggcggactcgtgaagcctggcggctctctgagactgagctgtgccgccagcggcttcaccttcaacacctacgccatgaactggatccggcaggcccctggcaagggcctggaatgggtgtcccggatcagaagcaagtacaacaattacgccacctactacgccgacagcgtgaaggaccggttcaccatcagccgggacaacgccaagaacagcctgtacctgcagatgaactccctgcgggccgaggacaccgccgtgtactattgtgtgcggcacggcaacttcggcaacagctatgtgtcttggtttgcctactggggccagggcaccctcgtgacagtctcgagcgcgtcgaccaaaggccccagcgtgttccctctggcccccagcagcaagagcacctctggcggaacagccgccctgggctgcctggtcaaggactacttccccgagcccgtgaccgtgtcctggaactctggcgccctgaccagcggcgtgcacacctttccagccgtgctccagagcagcggcctgtacagcctgagcagcgtcgtgaccgtgcccagcagcagcctgggcacccagacctacatctgcaacgtgaaccacaagcccagcaacacaaaggtggacaagcgggtggaacccaagagctgcgacaagacccacacctgtcccccctgccctgcccctgaactgctgggaggcccctccgtgttcctgttccccccaaagcctaaggacaccctgatgatcagccggacccccgaagtgacctgcgtggtggtggacgtgtcccacgaggaccctgaagtgaagtttaattggtacgtggacggcgtggaagtgcacaacgccaagaccaagcccagagaggaacagtacaacagcacctaccgggtggtgtccgtgctgaccgtgctgcaccaggactggctgaacggcaaagagtacaagtgcaaggtgtccaacaaggccctgcctgcccccatcgagaaaaccatcagcaaggccaaaggccagccccgcgagccccaggtgtacacactgccccctagccgggaagagatgaccaagaaccaggtgtccctgacctgcctcgtgaagggcttctaccccagcgacattgccgtggaatgggagagcaacggccagcccgagaacaactacaagaccaccccccctgtgctggacagcgacggctcattcttcctgtacagcaagctgaccgtggacaagagccggtggcagcagggcaacgtgttcagctgctccgtgatgcacgaggccctgcacaaccactacacccagaagtccctgagcctgagccccggcaagtga

SEQ ID NO: 43 - protein, 266 aa, Artificial Sequence
  source: /note="Description of Artificial Sequence: Synthetic polypeptide"
ASPAAPAPSAQAVVTQEPSLTVSPGGTVTLTCRSSTGAVTTSNYANWVQQKPGQAPRGLIGGTNKRAPWTPARFSGSLLGGKAALTITGAQAEDEADYYCALWYSNLWVFGGGTKLTVLGQASPAAPAPASPAAPAPASGSQVQLVESGGGLVKPGGSLRLSCAASGFTFNTYAMNWIRQAPGKGLEWVSRIRSKYNNYATYYADSVKDRFTISRDNAKNSLYLQMNSLRAEDTAVYYCVRHGNFGNSYVSWFAYWGQGTLVTVSS

SEQ ID NO: 44 - DNA, 798 bp, Artificial Sequence
  source: /note="Description of Artificial Sequence: Synthetic polynucleotide"
gcttctcctgctgctcctgctcctagcgctcaggccgtggttacacaagagcccagcctgacagttagccctggcggaacagtgaccctgacctgcagatcttctacaggcgccgtgaccaccagcaactacgccaattgggtgcagcagaagcctggacaggctcccagaggactgatcggcggcacaaacaaaagagccccttggacacccgccagattcagcggatcactgctcggaggaaaggccgcactgacaatcacaggtgcccaggccgaagatgaggccgattactattgcgccctgtggtacagcaacctgtgggtgttcggcggaggtaccaagctgaccgtgctgggccaggcctctcctgctgctcctgctccagcttctccagccgctccagctcctgctagcggatctcaggtgcagctggtggaatctggcggcggactcgtgaagcctggcggctctctgagactgagctgtgccgccagcggcttcaccttcaacacctacgccatgaactggatccggcaggcccctggcaagggcctggaatgggtgtcccggatcagaagcaagtacaacaattacgccacctactacgccgacagcgtgaaggaccggttcaccatcagccgggacaacgccaagaacagcctgtacctgcagatgaactccctgcgggccgaggacaccgccgtgtactattgtgtgcggcacggcaacttcggcaacagctatgtgtcttggtttgcctactggggccagggcaccctcgtgacagtctcgagc

SEQ ID NO: 45 - protein, 111 aa, Artificial Sequence; identical to SEQ ID NO: 13
  source: /note="Description of Artificial Sequence: Synthetic polypeptide"

SEQ ID NO: 46 - protein, 125 aa, Artificial Sequence; identical to SEQ ID NO: 9
  source: /note="Description of Artificial Sequence: Synthetic polypeptide"

SEQ ID NO: 47 - DNA, 333 bp, Artificial Sequence; identical to SEQ ID NO: 14
  source: /note="Description of Artificial Sequence: Synthetic polynucleotide"

SEQ ID NO: 48 - DNA, 375 bp, Artificial Sequence; identical to SEQ ID NO: 10
  source: /note="Description of Artificial Sequence: Synthetic polynucleotide"

SEQ ID NO: 49 - protein, 215 aa, Artificial Sequence
  source: /note="Description of Artificial Sequence: Synthetic polypeptide"
ELVVTQEPSLTVSPGGTVTLTCRSSTGAVTTSNYANWVQQKPGQAPRGLIGGTNKRAPGTPARFSGSLLGGKAALTLSGVQPEDEAEYYCALWYSNLWVFGGGTKLTVLGQPKAAPSVTLFPPSSEELQANKATLVCLISDFYPGAVTVAWKADSSPVKAGVETTTPSKQSNNKYAASSYLSLTPEQWKSHRSYSCQVTHEGSTVEKTVAPTECS

SEQ ID NO: 50 - protein, 455 aa, Artificial Sequence; identical to SEQ ID NO: 40
  source: /note="Description of Artificial Sequence: Synthetic polypeptide"

SEQ ID NO: 51 - DNA, 645 bp, Artificial Sequence
  source: /note="Description of Artificial Sequence: Synthetic polynucleotide"
gagctggtggtcacacaagagcccagcctgacagtttctcctggcggcacagtgaccctgacctgcagatcttctacaggcgccgtgaccacctccaactacgccaattgggtgcagcagaagcctggacaggctcccagaggactgatcggcggcacaaacaaaagagcccctggcacaccagccagattcagcggatcactgctcggaggaaaggccgctctgacactgtctggtgtccagcctgaagatgaggccgagtactactgcgccctgtggtacagcaatctgtgggtgttcggcggaggtaccaagctgaccgtgctgggccagcccaaagccgcccctagcgtgaccctgttccccccctcgagtgaggaactccaggccaacaaggccaccctcgtgtgcctgatcagcgacttctaccctggcgccgtgaccgtggcctggaaggccgatagcagccctgtgaaggccggcgtggaaaccaccacccccagcaagcagagcaacaacaaatacgccgccagcagctacctgagcctgacccccgagcagtggaagtcccacagatcctacagctgccaggtcacacacgagggcagcaccgtggaaaagaccgtggcccccaccgagtgcagc

SEQ ID NO: 52 - DNA, 1368 bp, Artificial Sequence; identical to SEQ ID NO: 42
  source: /note="Description of Artificial Sequence: Synthetic polynucleotide"

SEQ ID NO: 53 - protein, 266 aa, Artificial Sequence
  source: /note="Description of Artificial Sequence: Synthetic polypeptide"
ASPAAPAPSAELVVTQEPSLTVSPGGTVTLTCRSSTGAVTTSNYANWVQQKPGQAPRGLIGGTNKRAPGTPARFSGSLLGGKAALTLSGVQPEDEAEYYCALWYSNLWVFGGGTKLTVLGQASPAAPAPASPAAPAPASGSQVQLVESGGGLVKPGGSLRLSCAASGFTFNTYAMNWIRQAPGKGLEWVSRIRSKYNNYATYYADSVKDRFTISRDNAKNSLYLQMNSLRAEDTAVYYCVRHGNFGNSYVSWFAYWGQGTLVTVSS

SEQ ID NO: 54 - DNA, 798 bp, Artificial Sequence
  source: /note="Description of Artificial Sequence: Synthetic polynucleotide"
gcttctcctgctgctcctgctcctagcgctgagctggtggtcacacaagagcccagcctgacagtttctcctggcggcacagtgaccctgacctgcagatcttctacaggcgccgtgaccacctccaactacgccaattgggtgcagcagaagcctggacaggctcccagaggactgatcggcggcacaaacaaaagagcccctggcacaccagccagattcagcggatcactgctcggaggaaaggccgctctgacactgtctggtgtccagcctgaagatgaggccgagtactactgcgccctgtggtacagcaatctgtgggtgttcggcggaggtaccaagctgaccgtgctgggccaggcctctcctgctgctcctgctccagcttctccagccgctccagctcctgctagcggatctcaggtgcagctggtggaatctggcggcggactcgtgaagcctggcggctctctgagactgagctgtgccgccagcggcttcaccttcaacacctacgccatgaactggatccggcaggcccctggcaagggcctggaatgggtgtcccggatcagaagcaagtacaacaattacgccacctactacgccgacagcgtgaaggaccggttcaccatcagccgggacaacgccaagaacagcctgtacctgcagatgaactccctgcgggccgaggacaccgccgtgtactattgtgtgcggcacggcaacttcggcaacagctatgtgtcttggtttgcctactggggccagggcaccctcgtgacagtctcgagc

SEQ ID NO: 55 - protein, 111 aa, Artificial Sequence; identical to SEQ ID NO: 15
  source: /note="Description of Artificial Sequence: Synthetic polypeptide"

SEQ ID NO: 56 - protein, 125 aa, Artificial Sequence; identical to SEQ ID NO: 7
  source: /note="Description of Artificial Sequence: Synthetic polypeptide"

SEQ ID NO: 57 - DNA, 333 bp, Artificial Sequence; identical to SEQ ID NO: 16
  source: /note="Description of Artificial Sequence: Synthetic polynucleotide"

SEQ ID NO: 58 - DNA, 375 bp, Artificial Sequence; identical to SEQ ID NO: 8
  source: /note="Description of Artificial Sequence: Synthetic polynucleotide"

SEQ ID NO: 59 - protein, 215 aa, Artificial Sequence
  source: /note="Description of Artificial Sequence: Synthetic polypeptide"
QTVVTQEPSLTVSPGGTVTLTCRSSTGAVTTSNYANWVQQKPGQAPRGLIGGTNKRAPGTPARFSGSLLGGKAALTLLGAQPEDEAEYYCALWYSNLWVFGGGTKLTVLGQPKAAPSVTLFPPSSEELQANKATLVCLISDFYPGAVTVAWKADSSPVKAGVETTTPSKQSNNKYAASSYLSLTPEQWKSHRSYSCQVTHEGSTVEKTVAPTECS

SEQ ID NO: 60 - protein, 455 aa, Artificial Sequence
  source: /note="Description of Artificial Sequence: Synthetic polypeptide"
EVQLVESGGGLVKPGGSLRLSCAASGFTFNTYAMNWVRQAPGKGLEWVGRIRSKYNNYATYYADSVKDRFTISRDDSKNTLYLQMNSLKTEDTAVYYCTTHGNFGNSYVSWFAYWGQGTLVTVSSASTKGPSVFPLAPSSKSTSGGTAALGCLVKDYFPEPVTVSWNSGALTSGVHTFPAVLQSSGLYSLSSVVTVPSSSLGTQTYICNVNHKPSNTKVDKRVEPKSCDKTHTCPPCPAPELLGGPSVFLFPPKPKDTLMISRTPEVTCVVVDVSHEDPEVKFNWYVDGVEVHNAKTKPREEQYNSTYRVVSVLTVLHQDWLNGKEYKCKVSNKALPAPIEKTISKAKGQPREPQVYTLPPSREEMTKNQVSLTCLVKGFYPSDIAVEWESNGQPENNYKTTPPVLDSDGSFFLYSKLTVDKSRWQQGNVFSCSVMHEALHNHYTQKSLSLSPGK

SEQ ID NO: 61 - DNA, 645 bp, Artificial Sequence
  source: /note="Description of Artificial Sequence: Synthetic polynucleotide"
cagaccgtggtcacacaagagcccagcctgacagtttctcctggcggcacagtgaccctgacctgcagatcttctacaggcgccgtgaccaccagcaactacgccaattgggtgcagcagaagcctggacaggctcccagaggactgatcggcggcacaaacaaaagagcccctggcacaccagccagattcagcggatcactgctcggaggaaaggccgctctgacactgcttggagcacagcctgaagatgaggccgagtactactgcgccctgtggtacagcaatctgtgggtgttcggcggaggtaccaagctgaccgtgctgggccagcccaaagccgcccctagcgtgaccctgttccccccctcgagtgaggaactccaggccaacaaggccaccctcgtgtgcctgatcagcgacttctaccctggcgccgtgaccgtggcctggaaggccgatagcagccctgtgaaggccggcgtggaaaccaccacccccagcaagcagagcaacaacaaatacgccgccagcagctacctgagcctgacccccgagcagtggaagtcccacagatcctacagctgccaggtcacacacgagggcagcaccgtggaaaagaccgtggcccccaccgagtgcagc

SEQ ID NO: 62 - DNA, 1365 bp, Artificial Sequence
  source: /note="Description of Artificial Sequence: Synthetic polynucleotide"
gaagtgcagctggtggaatctggcggcggactcgtgaagcctggcggctctctgagactgagctgtgccgccagcggcttcaccttcaacacctacgccatgaactgggtgcgccaggcccctggcaaaggcctggaatgggtgggacggatcagaagcaagtacaacaattacgccacctactacgccgacagcgtgaaggaccggttcaccatcagccgggacgacagcaagaacaccctgtacctgcagatgaacagcctgaaaaccgaggacaccgccgtgtactactgcaccacccacggcaacttcggcaacagctatgtgtcttggtttgcctactggggccagggcaccctcgtgacagtctcgagcgcgtcgaccaaaggccccagcgtgttccctctggcccccagcagcaagagcacctctggcggaacagccgccctgggctgcctggtcaaggactacttccccgagcccgtgaccgtgtcctggaactctggcgccctgaccagcggcgtgcacacctttccagccgtgctccagagcagcggcctgtacagcctgagcagcgtcgtgaccgtgcccagcagcagcctgggcacccagacctacatctgcaacgtgaaccacaagcccagcaacacaaaggtggacaagcgggtggaacccaagagctgcgacaagacccacacctgtcccccctgccctgcccctgaactgctgggaggcccctccgtgttcctgttccccccaaagcctaaggacaccctgatgatcagccggacccccgaagtgacctgcgtggtggtggacgtgtcccacgaggaccctgaagtgaagtttaattggtacgtggacggcgtggaagtgcacaacgccaagaccaagcccagagaggaacagtacaacagcacctaccgggtggtgtccgtgctgaccgtgctgcaccaggactggctgaacggcaaagagtacaagtgcaaggtgtccaacaaggccctgcctgcccccatcgagaaaaccatcagcaaggccaaaggccagccccgcgagccccaggtgtacacactgccccctagccgggaagagatgaccaagaaccaggtgtccctgacctgcctcgtgaagggcttctaccccagcgacattgccgtggaatgggagagcaacggccagcccgagaacaactacaagaccaccccccctgtgctggacagcgacggctcattcttcctgtacagcaagctgaccgtggacaagagccggtggcagcagggcaacgtgttcagctgctccgtgatgcacgaggccctgcacaaccactacacccagaagtccctgagcctgagccccggcaag

SEQ ID NO: 63 - protein, 266 aa, Artificial Sequence
  source: /note="Description of Artificial Sequence: Synthetic polypeptide"
ASPAAPAPSAQTVVTQEPSLTVSPGGTVTLTCRSSTGAVTTSNYANWVQQKPGQAPRGLIGGTNKRAPGTPARFSGSLLGGKAALTLLGAQPEDEAEYYCALWYSNLWVFGGGTKLTVLGQASPAAPAPASPAAPAPASGSEVQLVESGGGLVKPGGSLRLSCAASGFTFNTYAMNWVRQAPGKGLEWVGRIRSKYNNYATYYADSVKDRFTISRDDSKNTLYLQMNSLKTEDTAVYYCTTHGNFGNSYVSWFAYWGQGTLVTVSS

SEQ ID NO: 64 - DNA, 798 bp, Artificial Sequence
  source: /note="Description of Artificial Sequence: Synthetic polynucleotide"
gcttctcctgctgctcctgctcctagcgctcagaccgtggtcacacaagagcccagcctgacagtttctcctggcggcacagtgaccctgacctgcagatcttctacaggcgccgtgaccaccagcaactacgccaattgggtgcagcagaagcctggacaggctcccagaggactgatcggcggcacaaacaaaagagcccctggcacaccagccagattcagcggatcactgctcggaggaaaggccgctctgacactgcttggagcacagcctgaagatgaggccgagtactactgcgccctgtggtacagcaatctgtgggtgttcggcggaggtaccaagctgaccgtgctgggccaggcctctcctgctgctcctgctccagcttctccagccgctccagctcctgctagcggatctgaagtgcagctggtggaatctggcggcggactcgtgaagcctggcggctctctgagactgagctgtgccgccagcggcttcaccttcaacacctacgccatgaactgggtgcgccaggcccctggcaaaggcctggaatgggtgggacggatcagaagcaagtacaacaattacgccacctactacgccgacagcgtgaaggaccggttcaccatcagccgggacgacagcaagaacaccctgtacctgcagatgaacagcctgaaaaccgaggacaccgccgtgtactactgcaccacccacggcaacttcggcaacagctatgtgtcttggtttgcctactggggccagggcaccctcgtgacagtctcgagc

SEQ ID NO: 65 - protein, 7 aa, Artificial Sequence
  source: /note="Description of Artificial Sequence: Synthetic peptide"
GTKFLAP

SEQ ID NO: 66 - DNA, 21 bp, Artificial Sequence
  source: /note="Description of Artificial Sequence: Synthetic oligonucleotide"
ggcacaaaatttctggcccct

SEQ ID NO: 67 - protein, 111 aa, Artificial Sequence; identical to SEQ ID NO: 17
  source: /note="Description of Artificial Sequence: Synthetic polypeptide"

SEQ ID NO: 68 - protein, 125 aa, Artificial Sequence; identical to SEQ ID NO: 7
  source: /note="Description of Artificial Sequence: Synthetic polypeptide"

SEQ ID NO: 69 - DNA, 333 bp, Artificial Sequence; identical to SEQ ID NO: 18
  source: /note="Description of Artificial Sequence: Synthetic polynucleotide"

SEQ ID NO: 70 - DNA, 375 bp, Artificial Sequence; identical to SEQ ID NO: 8
  source: /note="Description of Artificial Sequence: Synthetic polynucleotide"

SEQ ID NO: 71 - protein, 215 aa, Artificial Sequence
  source: /note="Description of Artificial Sequence: Synthetic polypeptide"
QTVVTQEPSLTVSPGGTVTLTCRSSTGAVTTSNYANWVQQKPGQAPRGLIGGTKFLAPGTPARFSGSLLGGKAALTLLGAQPEDEAEYYCALWYSNLWVFGGGTKLTVLGQPKAAPSVTLFPPSSEELQANKATLVCLISDFYPGAVTVAWKADSSPVKAGVETTTPSKQSNNKYAASSYLSLTPEQWKSHRSYSCQVTHEGSTVEKTVAPTECS

SEQ ID NO: 72 - protein, 455 aa, Artificial Sequence; identical to SEQ ID NO: 60
  source: /note="Description of Artificial Sequence: Synthetic polypeptide"

SEQ ID NO: 73 - DNA, 645 bp, Artificial Sequence
  source: /note="Description of Artificial Sequence: Synthetic polynucleotide"
cagaccgtggtcacacaagagcccagcctgacagtttctcctggcggcacagtgaccctgacctgcagatcttctacaggcgccgtgaccaccagcaactacgccaattgggtgcagcagaagcctggacaggctcccagaggactgatcggcggcacaaaatttctggcccctggcacaccagccagattctctggatctctgctcggcggaaaggccgctctgacactgcttggagcacagcctgaagatgaggccgagtactactgcgccctgtggtacagcaatctgtgggtgttcggcggaggtaccaagctgaccgtgctgggccagcccaaagccgcccctagcgtgaccctgttccccccctcgagtgaggaactccaggccaacaaggccaccctcgtgtgcctgatcagcgacttctaccctggcgccgtgaccgtggcctggaaggccgatagcagccctgtgaaggccggcgtggaaaccaccacccccagcaagcagagcaacaacaaatacgccgccagcagctacctgagcctgacccccgagcagtggaagtcccacagatcctacagctgccaggtcacacacgagggcagcaccgtggaaaagaccgtggcccccaccgagtgcagc

SEQ ID NO: 74 - DNA, 1365 bp, Artificial Sequence; identical to SEQ ID NO: 62
  source: /note="Description of Artificial Sequence: Synthetic polynucleotide"

SEQ ID NO: 75 - protein, 266 aa, Artificial Sequence
  source: /note="Description of Artificial Sequence: Synthetic polypeptide"
ASPAAPAPSAQTVVTQEPSLTVSPGGTVTLTCRSSTGAVTTSNYANWVQQKPGQAPRGLIGGTKFLAPGTPARFSGSLLGGKAALTLLGAQPEDEAEYYCALWYSNLWVFGGGTKLTVLGQASPAAPAPASPAAPAPASGSEVQLVESGGGLVKPGGSLRLSCAASGFTFNTYAMNWVRQAPGKGLEWVGRIRSKYNNYATYYADSVKDRFTISRDDSKNTLYLQMNSLKTEDTAVYYCTTHGNFGNSYVSWFAYWGQGTLVTVSS

SEQ ID NO: 76 - DNA, 798 bp, Artificial Sequence
  source: /note="Description of Artificial Sequence: Synthetic polynucleotide"
gcttctcctgctgctcctgctcctagcgctcagaccgtggtcacacaagagcccagcctgacagtttctcctggcggcacagtgaccctgacctgcagatcttctacaggcgccgtgaccaccagcaactacgccaattgggtgcagcagaagcctggacaggctcccagaggactgatcggcggcacaaaatttctggcccctggcacaccagccagattctctggatctctgctcggcggaaaggccgctctgacactgcttggagcacagcctgaagatgaggccgagtactactgcgccctgtggtacagcaatctgtgggtgttcggcggaggtaccaagctgaccgtgctgggccaggcctctcctgctgctcctgctccagcttctccagccgctccagctcctgctagcggatctgaagtgcagctggtggaatctggcggcggactcgtgaagcctggcggctctctgagactgagctgtgccgccagcggcttcaccttcaacacctacgccatgaactgggtgcgccaggcccctggcaaaggcctggaatgggtgggacggatcagaagcaagtacaacaattacgccacctactacgccgacagcgtgaaggaccggttcaccatcagccgggacgacagcaagaacaccctgtacctgcagatgaacagcctgaaaaccgaggacaccgccgtgtactactgcaccacccacggcaacttcggcaacagctatgtgtcttggtttgcctactggggccagggcaccctcgtgacagtctcgagc

SEQ ID NO: 77 - protein, 111 aa, Artificial Sequence; identical to SEQ ID NO: 19
  source: /note="Description of Artificial Sequence: Synthetic polypeptide"

SEQ ID NO: 78 - protein, 125 aa, Artificial Sequence; identical to SEQ ID NO: 7
  source: /note="Description of Artificial Sequence: Synthetic polypeptide"

SEQ ID NO: 79 - DNA, 333 bp, Artificial Sequence; identical to SEQ ID NO: 20
  source: /note="Description of Artificial Sequence: Synthetic polynucleotide"

SEQ ID NO: 80 - DNA, 375 bp, Artificial Sequence; identical to SEQ ID NO: 8
  source: /note="Description of Artificial Sequence: Synthetic polynucleotide"

SEQ ID NO: 81 - protein, 215 aa, Artificial Sequence
  source: /note="Description of Artificial Sequence: Synthetic polypeptide"
QTVVTQEPSLTVSPGGTVTLTCRSSTGAVTTSNYANWVQQKPGQAPRGLIGGTKFLAPGTPARFSGSLLGGKAALTLSGVQPEDEAEYYCALWYSNLWVFGGGTKLTVLGQPKAAPSVTLFPPSSEELQANKATLVCLISDFYPGAVTVAWKADSSPVKAGVETTTPSKQSNNKYAASSYLSLTPEQWKSHRSYSCQVTHEGSTVEKTVAPTECS

SEQ ID NO: 82 - protein, 455 aa, Artificial Sequence; identical to SEQ ID NO: 60
  source: /note="Description of Artificial Sequence: Synthetic polypeptide"

SEQ ID NO: 83 - DNA, 645 bp, Artificial Sequence
  source: /note="Description of Artificial Sequence: Synthetic polynucleotide"
cagaccgtggtcacacaagagcccagcctgacagtttctcctggcggcacagtgaccctgacctgcagatcttctacaggcgccgtgaccaccagcaactacgccaattgggtgcagcagaagcctggacaggctcccagaggactgatcggcggcacaaaatttctggcccctggcacaccagccagattctctggatctctgctcggcggaaaggccgctctgacactgtctggtgttcagcctgaggacgaggccgagtactattgcgccctgtggtacagcaacctgtgggtgttcggcggaggtaccaagctgaccgtgctgggccagcccaaagccgcccctagcgtgaccctgttccccccctcgagtgaggaactccaggccaacaaggccaccctcgtgtgcctgatcagcgacttctaccctggcgccgtgaccgtggcctggaaggccgatagcagccctgtgaaggccggcgtggaaaccaccacccccagcaagcagagcaacaacaaatacgccgccagcagctacctgagcctgacccccgagcagtggaagtcccacagatcctacagctgccaggtcacacacgagggcagcaccgtggaaaagaccgtggcccccaccgagtgcagc

SEQ ID NO: 84 - DNA, 1365 bp, Artificial Sequence; identical to SEQ ID NO: 62
  source: /note="Description of Artificial Sequence: Synthetic polynucleotide"

SEQ ID NO: 85 - protein, 111 aa, Artificial Sequence; identical to SEQ ID NO: 19
  source: /note="Description of Artificial Sequence: Synthetic polypeptide"

SEQ ID NO: 86 - protein, 125 aa, Artificial Sequence; identical to SEQ ID NO: 9
  source: /note="Description of Artificial Sequence: Synthetic polypeptide"

SEQ ID NO: 87 - DNA, 333 bp, Artificial Sequence; identical to SEQ ID NO: 20
  source: /note="Description of Artificial Sequence: Synthetic polynucleotide"

SEQ ID NO: 88 - DNA, 375 bp, Artificial Sequence; identical to SEQ ID NO: 10
  source: /note="Description of Artificial Sequence: Synthetic polynucleotide"

SEQ ID NO: 89 - protein, 215 aa, Artificial Sequence; identical to SEQ ID NO: 81
  source: /note="Description of Artificial Sequence: Synthetic polypeptide"

SEQ ID NO: 90 - protein, 455 aa, Artificial Sequence; identical to SEQ ID NO: 40
  source: /note="Description of Artificial Sequence: Synthetic polypeptide"

SEQ ID NO: 91 - DNA, 645 bp, Artificial Sequence; identical to SEQ ID NO: 83
  source: /note="Description of Artificial Sequence: Synthetic polynucleotide"

SEQ ID NO: 92 - DNA, 1368 bp, Artificial Sequence; identical to SEQ ID NO: 42
  source: /note="Description of Artificial Sequence: Synthetic polynucleotide"

SEQ ID NO: 93 - protein, 266 aa, Artificial Sequence
  source: /note="Description of Artificial Sequence: Synthetic polypeptide"
ASPAAPAPSAQTVVTQEPSLTVSPGGTVTLTCRSSTGAVTTSNYANWVQQKPGQAPRGLIGGTKFLAPGTPARFSGSLLGGKAALTLSGVQPEDEAEYYCALWYSNLWVFGGGTKLTVLGQASPAAPAPASPAAPAPASGSQVQLVESGGGLVKPGGSLRLSCAASGFTFNTYAMNWIRQAPGKGLEWVSRIRSKYNNYATYYADSVKDRFTISRDNAKNSLYLQMNSLRAEDTAVYYCVRHGNFGNSYVSWFAYWGQGTLVTVSS

SEQ ID NO: 94 - DNA, 798 bp, Artificial Sequence
  source: /note="Description of Artificial Sequence: Synthetic polynucleotide"
gcttctcctgctgctcctgctcctagcgctcagaccgtggtcacacaagagcccagcctgacagtttctcctggcggcacagtgaccctgacctgcagatcttctacaggcgccgtgaccaccagcaactacgccaattgggtgcagcagaagcctggacaggctcccagaggactgatcggcggcacaaaatttctggcccctggcacaccagccagattctctggatctctgctcggcggaaaggccgctctgacactgtctggtgttcagcctgaggacgaggccgagtactattgcgccctgtggtacagcaacctgtgggtgttcggcggaggtaccaagctgaccgtgctgggccaggcctctcctgctgctcctgctccagcttctccagccgctccagctcctgctagcggatctcaggtgcagctggtggaatctggcggcggactcgtgaagcctggcggctctctgagactgagctgtgccgccagcggcttcaccttcaacacctacgccatgaactggatccggcaggcccctggcaagggcctggaatgggtgtcccggatcagaagcaagtacaacaattacgccacctactacgccgacagcgtgaaggaccggttcaccatcagccgggacaacgccaagaacagcctgtacctgcagatgaactccctgcgggccgaggacaccgccgtgtactattgtgtgcggcacggcaacttcggcaacagctatgtgtcttggtttgcctactggggccagggcaccctcgtgacagtctcgagc

SEQ ID NO: 95 - protein, 111 aa, Artificial Sequence; identical to SEQ ID NO: 21
  source: /note="Description of Artificial Sequence: Synthetic polypeptide"

SEQ ID NO: 96 - protein, 125 aa, Artificial Sequence; identical to SEQ ID NO: 9
  source: /note="Description of Artificial Sequence: Synthetic polypeptide"

SEQ ID NO: 97 - DNA, 333 bp, Artificial Sequence; identical to SEQ ID NO: 22
  source: /note="Description of Artificial Sequence: Synthetic polynucleotide"

SEQ ID NO: 98 - DNA, 375 bp, Artificial Sequence; identical to SEQ ID NO: 10
  source: /note="Description of Artificial Sequence: Synthetic polynucleotide"

SEQ ID NO: 99 - protein, 215 aa, Artificial Sequence
  source: /note="Description of Artificial Sequence: Synthetic polypeptide"
QTVVTQEPSLTVSPGGTVTLTCRSSTGAVTTSNYANWVQQKPGQAPRGLIGGTNKRAPGTPARFSGSLLGGKAALTLSGVQPEDEAEYYCALWYSNLWVFGGGTKLTVLGQPKAAPSVTLFPPSSEELQANKATLVCLISDFYPGAVTVAWKADSSPVKAGVETTTPSKQSNNKYAASSYLSLTPEQWKSHRSYSCQVTHEGSTVEKTVAPTECS

SEQ ID NO: 100 - protein, 455 aa, Artificial Sequence; identical to SEQ ID NO: 40
  source: /note="Description of Artificial Sequence: Synthetic polypeptide"

SEQ ID NO: 101 - DNA, 645 bp, Artificial Sequence
  source: /note="Description of Artificial Sequence: Synthetic polynucleotide"
cagaccgtggtcacacaagagcccagcctgacagtttctcctggcggcacagtgaccctgacctgcagatcttctacaggcgccgtgaccaccagcaactacgccaattgggtgcagcagaagcctggacaggctcccagaggactgatcggcggcacaaacaaaagagcccctggcacaccagccagattcagcggatcactgctcggaggaaaggccgctctgacactgtctggtgtccagcctgaagatgaggccgagtactactgcgccctgtggtacagcaatctgtgggtgttcggcggaggtaccaagctgaccgtgctgggccagcccaaagccgcccctagcgtgaccctgttccccccctcgagtgaggaactccaggccaacaaggccaccctcgtgtgcctgatcagcgacttctaccctggcgccgtgaccgtggcctggaaggccgatagcagccctgtgaaggccggcgtggaaaccaccacccccagcaagcagagcaacaacaaatacgccgccagcagctacctgagcctgacccccgagcagtggaagtcccacagatcctacagctgccaggtcacacacgagggcagcaccgtggaaaagaccgtggcccccaccgagtgcagc

SEQ ID NO: 102 - DNA, 1368 bp, Artificial Sequence; identical to SEQ ID NO: 42
  source: /note="Description of Artificial Sequence: Synthetic polynucleotide"

SEQ ID NO: 103 - protein, 266 aa, Artificial Sequence
  source: /note="Description of Artificial Sequence: Synthetic polypeptide"
ASPAAPAPSAQTVVTQEPSLTVSPGGTVTLTCRSSTGAVTTSNYANWVQQKPGQAPRGLIGGTNKRAPGTPARFSGSLLGGKAALTLSGVQPEDEAEYYCALWYSNLWVFGGGTKLTVLGQASPAAPAPASPAAPAPASGSQVQLVESGGGLVKPGGSLRLSCAASGFTFNTYAMNWIRQAPGKGLEWVSRIRSKYNNYATYYADSVKDRFTISRDNAKNSLYLQMNSLRAEDTAVYYCVRHGNFGNSYVSWFAYWGQGTLVTVSS

SEQ ID NO: 104 - DNA, 798 bp, Artificial Sequence
  source: /note="Description of Artificial Sequence: Synthetic polynucleotide"
gcttctcctgctgctcctgctcctagcgctcagaccgtggtcacacaagagcccagcctgacagtttctcctggcggcacagtgaccctgacctgcagatcttctacaggcgccgtgaccaccagcaactacgccaattgggtgcagcagaagcctggacaggctcccagaggactgatcggcggcacaaacaaaagagcccctggcacaccagccagattcagcggatcactgctcggaggaaaggccgctctgacactgtctggtgtccagcctgaagatgaggccgagtactactgcgccctgtggtacagcaatctgtgggtgttcggcggaggtaccaagctgaccgtgctgggccaggcctctcctgctgctcctgctccagcttctccagccgctccagctcctgctagcggatctcaggtgcagctggtggaatctggcggcggactcgtgaagcctggcggctctctgagactgagctgtgccgccagcggcttcaccttcaacacctacgccatgaactggatccggcaggcccctggcaagggcctggaatgggtgtcccggatcagaagcaagtacaacaattacgccacctactacgccgacagcgtgaaggaccggttcaccatcagccgggacaacgccaagaacagcctgtacctgcagatgaactccctgcgggccgaggacaccgccgtgtactattgtgtgcggcacggcaacttcggcaacagctatgtgtcttggtttgcctactggggccagggcaccctcgtgacagtctcgagc

SEQ ID NO: 105 - protein, 716 aa, Artificial Sequence
  source: /note="Description of Artificial Sequence: Synthetic polypeptide"
QVQLVESGGGLVQPGGSLRLSCAASGFNIKDTYIHWVRQAPGKGLEWVARIYPTNGYTRYADSVKGRFTISADTSKNTAYLQMNSLRAEDTAVYYCSRWGGDGFYAMDYWGQGTLVTVSSASTKGPSVFPLAPSSKSTSGGTAALGCLVKDYFPEPVTVSWNSGALTSGVHTFPAVLQSSGLYSLSSVVTVPSSSLGTQTYICNVNHKPSNTKVDKRVEPKSCDKTHTCPPCPAPEAEGAPSVFLFPPKPKDTLMISRTPEVTCVVVDVSHEDPEVKFNWYVDGVEVHNAKTKPREEQYNSTYRVVSVLTVLHQDWLNGKEYKCKVSNKALPSSIEKTISKAKGQPREPQVYTLPPSREEMTKNQVSLTCLVKGFYPSDIAVEWESNGQPENNYKTTPPVLDSDGSFFLYSKLTVDKSRWQQGNVFSCSVMHEALHNHYTQKSLSLSPGKASPAAPAPSAQAVVTQEPSLTVSPGGTVTLTCRSSTGAVTTSNYANWVQQKPGQAPRGLIGGTNKRAPWTPARFSGSLLGGKAALTITGAQAEDEADYYCALWYSNLWVFGGGTKLTVLGQASPAAPAPASPAAPAPASGSQVQLVESGGGLVKPGGSLRLSCAASGFTFNTYAMNWIRQAPGKGLEWVSRIRSKYNNYATYYADSVKDRFTISRDNAKNSLYLQMNSLRAEDTAVYYCVRHGNFGNSYVSWFAYWGQGTLVTVSS

SEQ ID NO: 106 - DNA, 2148 bp, Artificial Sequence
  source: /note="Description of Artificial Sequence: Synthetic polynucleotide"
caggtgcaattggtggagtctggcggaggactggtgcagcctgggggcagcctgagactgagctgcgccgccagcggcttcaacatcaaggacacctacatccactgggtgcgccaggctccaggcaagggactggaatgggtggcccggatctaccccaccaacggctacaccagatacgccgacagcgtgaagggccggttcaccatcagcgccgacaccagcaagaacaccgcctacctgcagatgaacagcctgcgggccgaggacaccgccgtgtactactgcagcagatggggcggagatggcttctacgccatggactactggggccagggcaccctggtgaccgtctcgagcgcgtcgaccaaaggccccagcgtgttccctctggcccccagcagcaagagcacctctggcggaacagccgccctgggctgcctggtcaaggactacttccccgagcccgtgaccgtgtcctggaactctggcgccctgaccagcggcgtgcacacctttccagccgtgctccagagcagcggcctgtacagcctgagcagcgtcgtgaccgtgcccagcagcagcctgggcacccagacctacatctgcaacgtgaaccacaagcccagcaacacaaaggtggacaagcgggtggaacccaagagctgcgacaagacccacacctgtcccccctgccctgcccctgaagcggagggagccccctccgtgttcctgttccccccaaagcctaaggacaccctgatgatcagccggacccccgaagtgacctgcgtggtggtggacgtgtcccacgaggaccctgaagtgaagtttaattggtacgtggacggcgtggaagtgcacaacgccaagaccaagcccagagaggaacagtacaacagcacctaccgggtggtgtccgtgctgaccgtgctgcaccaggactggctgaacggcaaagagtacaagtgcaaggtgtccaacaaggccctgccttcctccatcgagaaaaccatcagcaaggccaaaggccagccccgcgagccccaggtgtacacactgccccctagccgggaagagatgaccaagaaccaggtgtccctgacctgcctcgtgaagggcttctaccccagcgacattgccgtggaatgggagagcaacggccagcccgagaacaactacaagaccaccccccctgtgctggacagcgacggctcattcttcctgtacagcaagctgaccgtggacaagagccggtggcagcagggcaacgtgttcagctgctccgtgatgcacgaggccctgcacaaccactacacccagaagtccctgagcctgagccccggcaaggcttctcctgctgctcctgctcctagcgctcaggccgtggttacacaagagcccagcctgacagttagccctggcggaacagtgaccctgacctgcagatcttctacaggcgccgtgaccaccagcaactacgccaattgggtgcagcagaagcctggacaggctcccagaggactgatcggcggcacaaacaaaagagccccttggacacccgccagattcagcggatcactgctcggaggaaaggccgcactgacaatcacaggtgcccaggccgaagatgaggccgattactattgcgccctgtggtacagcaacctgtgggtgttcggcggaggtaccaagctgaccgtgctgggccaggcctctcctgctgctcctgctccagcttctccagccgctccagctcctgctagcggatctcaggtgcagctggtggaatctggcggcggactcgtgaagcctggcggctctctgagactgagctgtgccgccagcggcttcaccttcaacacctacgccatgaactggatccggcaggcccctggcaagggcctggaatgggtgtcccggatcagaagcaagtacaacaattacgccacctactacgccgacagcgtgaaggaccggttcaccatcagccgggacaacgccaagaacagcctgtacctgcagatgaactccctgcgggccgaggacaccgccgtgtactattgtgtgcggcacggcaacttcggcaacagctatgtgtcttggtttgcctactggggccagggcaccctcgtgacagtctcgagc

SEQ ID NO: 107 - protein, 716 aa, Artificial Sequence
  source: /note="Description of Artificial Sequence: Synthetic polypeptide"
QVQLVESGGGLVQPGGSLRLSCAASGFNIKDTYIHWVRQAPGKGLEWVARIYPTNGYTRYADSVKGRFTISADTSKNTAYLQMNSLRAEDTAVYYCSRWGGDGFYAMDYWGQGTLVTVSSASTKGPSVFPLAPSSKSTSGGTAALGCLVKDYFPEPVTVSWNSGALTSGVHTFPAVLQSSGLYSLSSVVTVPSSSLGTQTYICNVNHKPSNTKVDKRVEPKSCDKTHTCPPCPAPEAEGAPSVFLFPPKPKDTLMISRTPEVTCVVVDVSHEDPEVKFNWYVDGVEVHNAKTKPREEQYNSTYRVVSVLTVLHQDWLNGKEYKCKVSNKALPSSIEKTISKAKGQPREPQVYTLPPSREEMTKNQVSLTCLVKGFYPSDIAVEWESNGQPENNYKTTPPVLDSDGSFFLYSKLTVDKSRWQQGNVFSCSVMHEALHNHYTQKSLSLSPGKASPAAPAPSAELVVTQEPSLTVSPGGTVTLTCRSSTGAVTTSNYANWVQQKPGQAPRGLIGGTNKRAPGTPARFSGSLLGGKAALTLSGVQPEDEAEYYCALWYSNLWVFGGGTKLTVLGQASPAAPAPASPAAPAPASGSQVQLVESGGGLVKPGGSLRLSCAASGFTFNTYAMNWIRQAPGKGLEWVSRIRSKYNNYATYYADSVKDRFTISRDNAKNSLYLQMNSLRAEDTAVYYCVRHGNFGNSYVSWFAYWGQGTLVTVSS

SEQ ID NO: 108 - DNA, 2148 bp, Artificial Sequence
  source: /note="Description of Artificial Sequence: Synthetic polynucleotide"
caggtgcaattggtggagtctggcggaggactggtgcagcctgggggcagcctgagactgagctgcgccgccagcggcttcaacatcaaggacacctacatccactgggtgcgccaggctccaggcaagggactggaatgggtggcccggatctaccccaccaacggctacaccagatacgccgacagcgtgaagggccggttcaccatcagcgccgacaccagcaagaacaccgcctacctgcagatgaacagcctgcgggccgaggacaccgccgtgtactactgcagcagatggggcggagatggcttctacgccatggactactggggccagggcaccctggtgaccgtctcgagcgcgtcgaccaaaggccccagcgtgttccctctggcccccagcagcaagagcacctctggcggaacagccgccctgggctgcctggtcaaggactacttccccgagcccgtgaccgtgtcctggaactctggcgccctgaccagcggcgtgcacacctttccagccgtgctccagagcagcggcctgtacagcctgagcagcgtcgtgaccgtgcccagcagcagcctgggcacccagacctacatctgcaacgtgaaccacaagcccagcaacacaaaggtggacaagcgggtggaacccaagagctgcgacaagacccacacctgtcccccctgccctgcccctgaagcggagggagccccctccgtgttcctgttccccccaaagcctaaggacaccctgatgatcagccggacccccgaagtgacctgcgtggtggtggacgtgtcccacgaggaccctgaagtgaagtttaattggtacgtggacggcgtggaagtgcacaacgccaagaccaagcccagagaggaacagtacaacagcacctaccgggtggtgtccgtgctgaccgtgctgcaccaggactggctgaacggcaaagagtacaagtgcaaggtgtccaacaaggccctgccttcctccatcgagaaaaccatcagcaaggccaaaggccagccccgcgagccccaggtgtacacactgccccctagccgggaagagatgaccaagaaccaggtgtccctgacctgcctcgtgaagggcttctaccccagcgacattgccgtggaatgggagagcaacggccagcccgagaacaactacaagaccaccccccctgtgctggacagcgacggctcattcttcctgtacagcaagctgaccgtggacaagagccggtggcagcagggcaacgtgttcagctgctccgtgatgcacgaggccctgcacaaccactacacccagaagtccctgagcctgagccccggcaaggcttctcctgctgctcctgctcctagcgctgagctggtggtcacacaagagcccagcctgacagtttctcctggcggcacagtgaccctgacctgcagatcttctacaggcgccgtgaccacctccaactacgccaattgggtgcagcagaagcctggacaggctcccagaggactgatcggcggcacaaacaaaagagcccctggcacaccagccagattcagcggatcactgctcggaggaaaggccgctctgacactgtctggtgtccagcctgaagatgaggccgagtactactgcgccctgtggtacagcaatctgtgggtgttcggcggaggtaccaagctgaccgtgctgggccaggcctctcctgctgctcctgctccagcttctccagccgctccagctcctgctagcggatctcaggtgcagctggtggaatctggcggcggactcgtgaagcctggcggctctctgagactgagctgtgccgccagcggcttcaccttcaacacctacgccatgaactggatccggcaggcccctggcaagggcctggaatgggtgtcccggatcagaagcaagtacaacaattacgccacctactacgccgacagcgtgaaggaccggttcaccatcagccgggacaacgccaagaacagcctgtacctgcagatgaactccctgcgggccgaggacaccgccgtgtactattgtgtgcggcacggcaacttcggcaacagctatgtgtcttggtttgcctactggggccagggcaccctcgtgacagtctcgagc

SEQ ID NO: 109 - protein, 716 aa, Artificial Sequence
  source: /note="Description of Artificial Sequence: Synthetic polypeptide"
QVQLVESGGGLVQPGGSLRLSCAASGFNIKDTYIHWVRQAPGKGLEWVARIYPTNGYTRYADSVKGRFTISADTSKNTAYLQMNSLRAEDTAVYYCSRWGGDGFYAMDYWGQGTLVTVSSASTKGPSVFPLAPSSKSTSGGTAALGCLVKDYFPEPVTVSWNSGALTSGVHTFPAVLQSSGLYSLSSVVTVPSSSLGTQTYICNVNHKPSNTKVDKRVEPKSCDKTHTCPPCPAPEAEGAPSVFLFPPKPKDTLMISRTPEVTCVVVDVSHEDPEVKFNWYVDGVEVHNAKTKPREEQYNSTYRVVSVLTVLHQDWLNGKEYKCKVSNKALPSSIEKTISKAKGQPREPQVYTLPPSREEMTKNQVSLTCLVKGFYPSDIAVEWESNGQPENNYKTTPPVLDSDGSFFLYSKLTVDKSRWQQGNVFSCSVMHEALHNHYTQKSLSLSPGKASPAAPAPSAQTVVTQEPSLTVSPGGTVTLTCRSSTGAVTTSNYANWVQQKPGQAPRGLIGGTNKRAPGTPARFSGSLLGGKAALTLLGAQPEDEAEYYCALWYSNLWVFGGGTKLTVLGQASPAAPAPASPAAPAPASGSEVQLVESGGGLVKPGGSLRLSCAASGFTFNTYAMNWVRQAPGKGLEWVGRIRSKYNNYATYYADSVKDRFTISRDDSKNTLYLQMNSLKTEDTAVYYCTTHGNFGNSYVSWFAYWGQGTLVTVSS

SEQ ID NO: 110 - DNA, 2148 bp, Artificial Sequence
  source: /note="Description of Artificial Sequence: Synthetic polynucleotide"
caggtgcaattggtggagtctggcggaggactggtgcagcctgggggcagcctgagactgagctgcgccgccagcggcttcaacatcaaggacacctacatccactgggtgcgccaggctccaggcaagggactggaatgggtggcccggatctaccccaccaacggctacaccagatacgccgacagcgtgaagggccggttcaccatcagcgccgacaccagcaagaacaccgcctacctgcagatgaacagcctgcgggccgaggacaccgccgtgtactactgcagcagatggggcggagatggcttctacgccatggactactggggccagggcaccctggtgaccgtctcgagcgcgtcgaccaaaggccccagcgtgttccctctggcccccagcagcaagagcacctctggcggaacagccgccctgggctgcctggtcaaggactacttccccgagcccgtgaccgtgtcctggaactctggcgccctgaccagcggcgtgcacacctttccagccgtgctccagagcagcggcctgtacagcctgagcagcgtcgtgaccgtgcccagcagcagcctgggcacccagacctacatctgcaacgtgaaccacaagcccagcaacacaaaggtggacaagcgggtggaacccaagagctgcgacaagacccacacctgtcccccctgccctgcccctgaagcggagggagccccctccgtgttcctgttccccccaaagcctaaggacaccctgatgatcagccggacccccgaagtgacctgcgtggtggtggacgtgtcccacgaggaccctgaagtgaagtttaattggtacgtggacggcgtggaagtgcacaacgccaagaccaagcccagagaggaacagtacaacagcacctaccgggtggtgtccgtgctgaccgtgctgcaccaggactggctgaacggcaaagagtacaagtgcaaggtgtccaacaaggccctgccttcctccatcgagaaaaccatcagcaaggccaaaggccagccccgcgagccccaggtgtacacactgccccctagccgggaagagatgaccaagaaccaggtgtccctgacctgcctcgtgaagggcttctaccccagcgacattgccgtggaatgggagagcaacggccagcccgagaacaactacaagaccaccccccctgtgctggacagcgacggctcattcttcctgtacagcaagctgaccgtggacaagagccggtggcagcagggcaacgtgttcagctgctccgtgatgcacgaggccctgcacaaccactacacccagaagtccctgagcctgagccccggcaaggcttctcctgctgctcctgctcctagcgctcagaccgtggtcacacaagagcccagcctgacagtttctcctggcggcacagtgaccctgacctgcagatcttctacaggcgccgtgaccaccagcaactacgccaattgggtgcagcagaagcctggacaggctcccagaggactgatcggcggcacaaacaaaagagcccctggcacaccagccagattcagcggatcactgctcggaggaaaggccgctctgacactgcttggagcacagcctgaagatgaggccgagtactactgcgccctgtggtacagcaatctgtgggtgttcggcggaggtaccaagctgaccgtgctgggccaggcctctcctgctgctcctgctccagcttctccagccgctccagctcctgctagcggatctgaagtgcagctggtggaatctggcggcggactcgtgaagcctggcggctctctgagactgagctgtgccgccagcggcttcaccttcaacacctacgccatgaactgggtgcgccaggcccctggcaaaggcctggaatgggtgggacggatcagaagcaagtacaacaattacgccacctactacgccgacagcgtgaaggaccggttcaccatcagccgggacgacagcaagaacaccctgtacctgcagatgaacagcctgaaaaccgaggacaccgccgtgtactactgcaccacccacggcaacttcggcaacagctatgtgtcttggtttgcctactggggccagggcaccctcgtgacagtctcgagc

SEQ ID NO: 111 - protein, 716 aa, Artificial Sequence
  source: /note="Description of Artificial Sequence: Synthetic polypeptide"
QVQLVESGGGLVQPGGSLRLSCAASGFNIKDTYIHWVRQAPGKGLEWVARIYPTNGYTRYADSVKGRFTISADTSKNTAYLQMNSLRAEDTAVYYCSRWGGDGFYAMDYWGQGTLVTVSSASTKGPSVFPLAPSSKSTSGGTAALGCLVKDYFPEPVTVSWNSGALTSGVHTFPAVLQSSGLYSLSSVVTVPSSSLGTQTYICNVNHKPSNTKVDKRVEPKSCDKTHTCPPCPAPEAEGAPSVFLFPPKPKDTLMISRTPEVTCVVVDVSHEDPEVKFNWYVDGVEVHNAKTKPREEQYNSTYRVVSVLTVLHQDWLNGKEYKCKVSNKALPSSIEKTISKAKGQPREPQVYTLPPSREEMTKNQVSLTCLVKGFYPSDIAVEWESNGQPENNYKTTPPVLDSDGSFFLYSKLTVDKSRWQQGNVFSCSVMHEALHNHYTQKSLSLSPGKASPAAPAPSAQTVVTQEPSLTVSPGGTVTLTCRSSTGAVTTSNYANWVQQKPGQAPRGLIGGTKFLAPGTPARFSGSLLGGKAALTLLGAQPEDEAEYYCALWYSNLWVFGGGTKLTVLGQASPAAPAPASPAAPAPASGSEVQLVESGGGLVKPGGSLRLSCAASGFTFNTYAMNWVRQAPGKGLEWVGRIRSKYNNYATYYADSVKDRFTISRDDSKNTLYLQMNSLKTEDTAVYYCTTHGNFGNSYVSWFAYWGQGTLVTVSS

SEQ ID NO: 112 - DNA, 2148 bp, Artificial Sequence
  source: /note="Description of Artificial Sequence: Synthetic polynucleotide"
caggtgcaattggtggagtctggcggaggactggtgcagcctgggggcagcctgagactgagctgcgccgccagcggcttcaacatcaaggacacctacatccactgggtgcgccaggctccaggcaagggactggaatgggtggcccggatctaccccaccaacggctacaccagatacgccgacagcgtgaagggccggttcaccatcagcgccgacaccagcaagaacaccgcctacctgcagatgaacagcctgcgggccgaggacaccgccgtgtactactgcagcagatggggcggagatggcttctacgccatggactactggggccagggcaccctggtgaccgtctcgagcgcgtcgaccaaaggccccagcgtgttccctctggcccccagcagcaagagcacctctggcggaacagccgccctgggctgcctggtcaaggactacttccccgagcccgtgaccgtgtcctggaactctggcgccctgaccagcggcgtgcacacctttccagccgtgctccagagcagcggcctgtacagcctgagcagcgtcgtgaccgtgcccagcagcagcctgggcacccagacctacatctgcaacgtgaaccacaagcccagcaacacaaaggtggacaagcgggtggaacccaagagctgcgacaagacccacacctgtcccccctgccctgcccctgaagcggagggagccccctccgtgttcctgttccccccaaagcctaaggacaccctgatgatcagccggacccccgaagtgacctgcgtggtggtggacgtgtcccacgaggaccctgaagtgaagtttaattggtacgtggacggcgtggaagtgcacaacgccaagaccaagcccagagaggaacagtacaacagcacctaccgggtggtgtccgtgctgaccgtgctgcaccaggactggctgaacggcaaagagtacaagtgcaaggtgtccaacaaggccctgccttcctccatcgagaaaaccatcagcaaggccaaaggccagccccgcgagccccaggtgtacacactgccccctagccgggaagagatgaccaagaaccaggtgtccctgacctgcctcgtgaagggcttctaccccagcgacattgccgtggaatgggagagcaacggccagcccgagaacaactacaagaccaccccccctgtgctggacagcgacggctcattcttcctgtacagcaagctgaccgtggacaagagccggtggcagcagggcaacgtgttcagctgctccgtgatgcacgaggccctgcacaaccactacacccagaagtccctgagcctgagccccggcaaggcttctcctgctgctcctgctcctagcgctcagaccgtggtcacacaagagcccagcctgacagtttctcctggcggcacagtgaccctgacctgcagatcttctacaggcgccgtgaccaccagcaactacgccaattgggtgcagcagaagcctggacaggctcccagaggactgatcggcggcacaaaatttctggcccctggcacaccagccagattctctggatctctgctcggcggaaaggccgctctgacactgcttggagcacagcctgaagatgaggccgagtactactgcgccctgtggtacagcaatctgtgggtgttcggcggaggtaccaagctgaccgtgctgggccaggcctctcctgctgctcctgctccagcttctccagccgctccagctcctgctagcggatctgaagtgcagctggtggaatctggcggcggactcgtgaagcctggcggctctctgagactgagctgtgccgccagcggcttcaccttcaacacctacgccatgaactgggtgcgccaggcccctggcaaaggcctggaatgggtgggacggatcagaagcaagtacaacaattacgccacctactacgccgacagcgtgaaggaccggttcaccatcagccgggacgacagcaagaacaccctgtacctgcagatgaacagcctgaaaaccgaggacaccgccgtgtactactgcaccacccacggcaacttcggcaacagctatgtgtcttggtttgcctactggggccagggcaccctcgtgacagtctcgagc

SEQ ID NO: 113 - protein, 716 aa, Artificial Sequence
  source: /note="Description of Artificial Sequence: Synthetic polypeptide"
QVQLVESGGGLVQPGGSLRLSCAASGFNIKDTYIHWVRQAPGKGLEWVARIYPTNGYTRYADSVKGRFTISADTSKNTAYLQMNSLRAEDTAVYYCSRWGGDGFYAMDYWGQGTLVTVSSASTKGPSVFPLAPSSKSTSGGTAALGCLVKDYFPEPVTVSWNSGALTSGVHTFPAVLQSSGLYSLSSVVTVPSSSLGTQTYICNVNHKPSNTKVDKRVEPKSCDKTHTCPPCPAPEAEGAPSVFLFPPKPKDTLMISRTPEVTCVVVDVSHEDPEVKFNWYVDGVEVHNAKTKPREEQYNSTYRVVSVLTVLHQDWLNGKEYKCKVSNKALPSSIEKTISKAKGQPREPQVYTLPPSREEMTKNQVSLTCLVKGFYPSDIAVEWESNGQPENNYKTTPPVLDSDGSFFLYSKLTVDKSRWQQGNVFSCSVMHEALHNHYTQKSLSLSPGKASPAAPAPSAQTVVTQEPSLTVSPGGTVTLTCRSSTGAVTTSNYANWVQQKPGQAPRGLIGGTKFLAPGTPARFSGSLLGGKAALTLSGVQPEDEAEYYCALWYSNLWVFGGGTKLTVLGQASPAAPAPASPAAPAPASGSEVQLVESGGGLVKPGGSLRLSCAASGFTFNTYAMNWVRQAPGKGLEWVGRIRSKYNNYATYYADSVKDRFTISRDDSKNTLYLQMNSLKTEDTAVYYCTTHGNFGNSYVSWFAYWGQGTLVTVSS

SEQ ID NO: 114 - DNA, 2148 bp, Artificial Sequence
  source: /note="Description of Artificial Sequence: Synthetic polynucleotide"
caggtgcaattggtggagtctggcggaggactggtgcagcctgggggcagcctgagactgagctgcgccgccagcggcttcaacatcaaggacacctacatccactgggtgcgccaggctccaggcaagggactggaatgggtggcccggatctaccccaccaacggctacaccagatacgccgacagcgtgaagggccggttcaccatcagcgccgacaccagcaagaacaccgcctacctgcagatgaacagcctgcgggccgaggacaccgccgtgtactactgcagcagatggggcggagatggcttctacgccatggactactggggccagggcaccctggtgaccgtctcgagcgcgtcgaccaaaggccccagcgtgttccctctggcccccagcagcaagagcacctctggcggaacagccgccctgggctgcctggtcaaggactacttccccgagcccgtgaccgtgtcctggaactctggcgccctgaccagcggcgtgcacacctttccagccgtgctccagagcagcggcctgtacagcctgagcagcgtcgtgaccgtgcccagcagcagcctgggcacccagacctacatctgcaacgtgaaccacaagcccagcaacacaaaggtggacaagcgggtggaacccaagagctgcgacaagacccacacctgtcccccctgccctgcccctgaagcggagggagccccctccgtgttcctgttccccccaaagcctaaggacaccctgatgatcagccggacccccgaagtgacctgcgtggtggtggacgtgtcccacgaggaccctgaagtgaagtttaattggtacgtggacggcgtggaagtgcacaacgccaagaccaagcccagagaggaacagtacaacagcacctaccgggtggtgtccgtgctgaccgtgctgcaccaggactggctgaacggcaaagagtacaagtgcaaggtgtccaacaaggccctgccttcctccatcgagaaaaccatcagcaaggccaaaggccagccccgcgagccccaggtgtacacactgccccctagccgggaagagatgaccaagaaccaggtgtccctgacctgcctcgtgaagggcttctaccccagcgacattgccgtggaatgggagagcaacggccagcccgagaacaactacaagaccaccccccctgtgctggacagcgacggctcattcttcctgtacagcaagctgaccgtggacaagagccggtggcagcagggcaacgtgttcagctgctccgtgatgcacgaggccctgcacaaccactacacccagaagtccctgagcctgagccccggcaaggcttctcctgctgctcctgctcctagcgctcagaccgtggtcacacaagagcccagcctgacagtttctcctggcggcacagtgaccctgacctgcagatcttctacaggcgccgtgaccaccagcaactacgccaattgggtgcagcagaagcctggacaggctcccagaggactgatcggcggcacaaaatttctggcccctggcacaccagccagattctctggatctctgctcggcggaaaggccgctctgacactgtctggtgttcagcctgaggacgaggccgagtactattgcgccctgtggtacagcaacctgtgggtgttcggcggaggtaccaagctgaccgtgctgggccaggcctctcctgctgctcctgctccagcttctccagccgctccagctcctgctagcggatctgaagtgcagctggtggaatctggcggcggactcgtgaagcctggcggctctctgagactgagctgtgccgccagcggcttcaccttcaacacctacgccatgaactgggtgcgccaggcccctggcaaaggcctggaatgggtgggacggatcagaagcaagtacaacaattacgccacctactacgccgacagcgtgaaggaccggttcaccatcagccgggacgacagcaagaacaccctgtacctgcagatgaacagcctgaaaaccgaggacaccgccgtgtactactgcaccacccacggcaacttcggcaacagctatgtgtcttggtttgcctactggggccagggcaccctcgtgacagtctcgagc

SEQ ID NO: 115 - protein, 716 aa, Artificial Sequence
  source: /note="Description of Artificial Sequence: Synthetic polypeptide"
QVQLVESGGGLVQPGGSLRLSCAASGFNIKDTYIHWVRQAPGKGLEWVARIYPTNGYTRYADSVKGRFTISADTSKNTAYLQMNSLRAEDTAVYYCSRWGGDGFYAMDYWGQGTLVTVSSASTKGPSVFPLAPSSKSTSGGTAALGCLVKDYFPEPVTVSWNSGALTSGVHTFPAVLQSSGLYSLSSVVTVPSSSLGTQTYICNVNHKPSNTKVDKRVEPKSCDKTHTCPPCPAPEAEGAPSVFLFPPKPKDTLMISRTPEVTCVVVDVSHEDPEVKFNWYVDGVEVHNAKTKPREEQYNSTYRVVSVLTVLHQDWLNGKEYKCKVSNKALPSSIEKTISKAKGQPREPQVYTLPPSREEMTKNQVSLTCLVKGFYPSDIAVEWESNGQPENNYKTTPPVLDSDGSFFLYSKLTVDKSRWQQGNVFSCSVMHEALHNHYTQKSLSLSPGKASPAAPAPSAQTVVTQEPSLTVSPGGTVTLTCRSSTGAVTTSNYANWVQQKPGQAPRGLIGGTKFLAPGTPARFSGSLLGGKAALTLSGVQPEDEAEYYCALWYSNLWVFGGGTKLTVLGQASPAAPAPASPAAPAPASGSQVQLVESGGGLVKPGGSLRLSCAASGFTFNTYAMNWIRQAPGKGLEWVSRIRSKYNNYATYYADSVKDRFTISRDNAKNSLYLQMNSLRAEDTAVYYCVRHGNFGNSYVSWFAYWGQGTLVTVSS

SEQ ID NO: 116 - DNA, 2148 bp, Artificial Sequence
  source: /note="Description of Artificial Sequence: Synthetic polynucleotide"
caggtgcaattggtggagtctggcggaggactggtgcagcctgggggcagcctgagactgagctgcgccgccagcggcttcaacatcaaggacacctacatccactgggtgcgccaggctccaggcaagggactggaatgggtggcccggatctaccccaccaacggctacaccagatacgccgacagcgtgaagggccggttcaccatcagcgccgacaccagcaagaacaccgcctacctgcagatgaacagcctgcgggccgaggacaccgccgtgtactactgcagcagatggggcggagatggcttctacgccatggactactggggccagggcaccctggtgaccgtctcgagcgcgtcgaccaaaggccccagcgtgttccctctggcccccagcagcaagagcacctctggcggaacagccgccctgggctgcctggtcaaggactacttccccgagcccgtgaccgtgtcctggaactctggcgccctgaccagcggcgtgcacacctttccagccgtgctccagagcagcggcctgtacagcctgagcagcgtcgtgaccgtgcccagcagcagcctgggcacccagacctacatctgcaacgtgaaccacaagcccagcaacacaaaggtggacaagcgggtggaacccaagagctgcgacaagacccacacctgtcccccctgccctgcccctgaagcggagggagccccctccgtgttcctgttccccccaaagcctaaggacaccctgatgatcagccggacccccgaagtgacctgcgtggtggtggacgtgtcccacgaggaccctgaagtgaagtttaattggtacgtggacggcgtggaagtgcacaacgccaagaccaagcccagagaggaacagtacaacagcacctaccgggtggtgtccgtgctgaccgtgctgcaccaggactggctgaacggcaaagagtacaagtgcaaggtgtccaacaaggccctgccttcctccatcgagaaaaccatcagcaaggccaaaggccagccccgcgagccccaggtgtacacactgccccctagccgggaagagatgaccaagaaccaggtgtccctgacctgcctcgtgaagggcttctaccccagcgacattgccgtggaatgggagagcaacggccagcccgagaacaactacaagaccaccccccctgtgctggacagcgacggctcattcttcctgtacagcaagctgaccgtggacaagagccggtggcagcagggcaacgtgttcagctgctccgtgatgcacgaggccctgcacaaccactacacccagaagtccctgagcctgagccccggcaaggcttctcctgctgctcctgctcctagcgctcagaccgtggtcacacaagagcccagcctgacagtttctcctggcggcacagtgaccctgacctgcagatcttctacaggcgccgtgaccaccagcaactacgccaattgggtgcagcagaagcctggacaggctcccagaggactgatcggcggcacaaaatttctggcccctggcacaccagccagattctctggatctctgctcggcggaaaggccgctctgacactgtctggtgttcagcctgaggacgaggccgagtactattgcgccctgtggtacagcaacctgtgggtgttcggcggaggtaccaagctgaccgtgctgggccaggcctctcctgctgctcctgctccagcttctccagccgctccagctcctgctagcggatctcaggtgcagctggtggaatctggcggcggactcgtgaagcctggcggctctctgagactgagctgtgccgccagcggcttcaccttcaacacctacgccatgaactggatccggcaggcccctggcaagggcctggaatgggtgtcccggatcagaagcaagtacaacaattacgccacctactacgccgacagcgtgaaggaccggttcaccatcagccgggacaacgccaagaacagcctgtacctgcagatgaactccctgcgggccgaggacaccgccgtgtactattgtgtgcggcacggcaacttcggcaacagctatgtgtcttggtttgcctactggggccagggcaccctcgtgacagtctcgagc

SEQ ID NO: 117 - protein, 716 aa, Artificial Sequence
  source: /note="Description of Artificial Sequence: Synthetic polypeptide"
QVQLVESGGGLVQPGGSLRLSCAASGFNIKDTYIHWVRQAPGKGLEWVARIYPTNGYTRYADSVKGRFTISADTSKNTAYLQMNSLRAEDTAVYYCSRWGGDGFYAMDYWGQGTLVTVSSASTKGPSVFPLAPSSKSTSGGTAALGCLVKDYFPEPVTVSWNSGALTSGVHTFPAVLQSSGLYSLSSVVTVPSSSLGTQTYICNVNHKPSNTKVDKRVEPKSCDKTHTCPPCPAPEAEGAPSVFLFPPKPKDTLMISRTPEVTCVVVDVSHEDPEVKFNWYVDGVEVHNAKTKPREEQYNSTYRVVSVLTVLHQDWLNGKEYKCKVSNKALPSSIEKTISKAKGQPREPQVYTLPPSREEMTKNQVSLTCLVKGFYPSDIAVEWESNGQPENNYKTTPPVLDSDGSFFLYSKLTVDKSRWQQGNVFSCSVMHEALHNHYTQKSLSLSPGKASPAAPAPSAQTVVTQEPSLTVSPGGTVTLTCRSSTGAVTTSNYANWVQQKPGQAPRGLIGGTNKRAPGTPARFSGSLLGGKAALTLSGVQPEDEAEYYCALWYSNLWVFGGGTKLTVLGQASPAAPAPASPAAPAPASGSQVQLVESGGGLVKPGGSLRLSCAASGFTFNTYAMNWIRQAPGKGLEWVSRIRSKYNNYATYYADSVKDRFTISRDNAKNSLYLQMNSLRAEDTAVYYCVRHGNFGNSYVSWFAYWGQGTLVTVSS

SEQ ID NO: 118 - DNA, 2148 bp, Artificial Sequence
  source: /note="Description of Artificial Sequence: Synthetic polynucleotide"
caggtgcaattggtggagtctggcggaggactggtgcagcctgggggcagcctgagactgagctgcgccgccagcggcttcaacatcaaggacacctacatccactgggtgcgccaggctccaggcaagggactggaatgggtggcccggatctaccccaccaacggctacaccagatacgccgacagcgtgaagggccggttcaccatcagcgccgacaccagcaagaacaccgcctacctgcagatgaacagcctgcgggccgaggacaccgccgtgtactactgcagcagatggggcggagatggcttctacgccatggactactggggccagggcaccctggtgaccgtctcgagcgcgtcgaccaaaggccccagcgtgttccctctggcccccagcagcaagagcacctctggcggaacagccgccctgggctgcctggtcaaggactacttccccgagcccgtgaccgtgtcctggaactctggcgccctgaccagcggcgtgcacacctttccagccgtgctccagagcagcggcctgtacagcctgagcagcgtcgtgaccgtgcccagcagcagcctgggcacccagacctacatctgcaacgtgaaccacaagcccagcaacacaaaggtggacaagcgggtggaacccaagagctgcgacaagacccacacctgtcccccctgccctgcccctgaagcggagggagccccctccgtgttcctgttccccccaaagcctaaggacaccctgatgatcagccggacccccgaagtgacctgcgtggtggtggacgtgtcccacgaggaccctgaagtgaagtttaattggtacgtggacggcgtggaagtgcacaacgccaagaccaagcccagagaggaacagtacaacagcacctaccgggtggtgtccgtgctgaccgtgctgcaccaggactggctgaacggcaaagagtacaagtgcaaggtgtccaacaaggccctgccttcctccatcgagaaaaccatcagcaaggccaaaggccagccccgcgagccccaggtgtacacactgccccctagccgggaagagatgaccaagaaccaggtgtccctgacctgcctcgtgaagggcttctaccccagcgacattgccgtggaatgggagagcaacggccagcccgagaacaactacaagaccaccccccctgtgctggacagcgacggctcattcttcctgtacagcaagctgaccgtggacaagagccggtggcagcagggcaacgtgttcagctgctccgtgatgcacgaggccctgcacaaccactacacccagaagtccctgagcctgagccccggcaaggcttctcctgctgctcctgctcctagcgctcagaccgtggtcacacaagagcccagcctgacagtttctcctggcggcacagtgaccctgacctgcagatcttctacaggcgccgtgaccaccagcaactacgccaattgggtgcagcagaagcctggacaggctcccagaggactgatcggcggcacaaacaaaagagcccctggcacaccagccagattcagcggatcactgctcggaggaaaggccgctctgacactgtctggtgtccagcctgaagatgaggccgagtactactgcgccctgtggtacagcaatctgtgggtgttcggcggaggtaccaagctgaccgtgctgggccaggcctctcctgctgctcctgctccagcttctccagccgctccagctcctgctagcggatctcaggtgcagctggtggaatctggcggcggactcgtgaagcctggcggctctctgagactgagctgtgccgccagcggcttcaccttcaacacctacgccatgaactggatccggcaggcccctggcaagggcctggaatgggtgtcccggatcagaagcaagtacaacaattacgccacctactacgccgacagcgtgaaggaccggttcaccatcagccgggacaacgccaagaacagcctgtacctgcagatgaactccctgcgggccgaggacaccgccgtgtactattgtgtgcggcacggcaacttcggcaacagctatgtgtcttggtttgcctactggggccagggcaccctcgtgacagtctcgagc

SEQ ID NO: 119 - protein, 214 aa, Artificial Sequence
  source: /note="Description of Artificial Sequence: Synthetic polypeptide"
DIQMTQSPSSLSASVGDRVTITCRASQDVNTAVAWYQQKPGKAPKLLIYSASFLYSGVPSRFSGSRSGTDFTLTISSLQPEDFATYYCQQHYTTPPTFGQGTKVEIKRTVAAPSVFIFPPSDEQLKSGTASVVCLLNNFYPREAKVQWKVDNALQSGNSQESVTEQDSKDSTYSLSSTLTLSKADYEKHKVYACEVTHQGLSSPVTKSFNRGEC

SEQ ID NO: 120 - DNA, 642 bp, Artificial Sequence
  source: /note="Description of Artificial Sequence: Synthetic polynucleotide"
gatatccagatgacccagagccccagcagcctgagcgccagcgtgggcgacagagtgaccatcacctgccgggccagccaggacgtgaacaccgccgtggcctggtatcagcagaagcccggcaaggcccccaagctgctgatctacagcgccagcttcctgtacagcggcgtgcccagccggttcagcggcagcagaagcggcaccgacttcaccctgaccatcagctccctgcagcccgaggacttcgccacctactactgccagcagcactacaccaccccccccaccttcggccagggtaccaaagtggaaatcaagcggaccgtggccgctccctccgtgttcatcttcccacccagcgacgagcagctgaagtccggcacagccagcgtcgtgtgcctgctgaacaacttctacccccgcgaggccaaagtgcagtggaaggtggacaacgccctccagagcggcaacagccaggaaagcgtcaccgagcaggacagcaaggactccacctacagcctgagcagcaccctgaccctgagcaaggccgactacgagaagcacaaggtgtacgcctgcgaagtgacccaccagggcctgtccagccccgtgaccaagagcttcaaccggggcgagtgt

SEQ ID NO: 121 - protein, 714 aa, Artificial Sequence
  source: /note="Description of Artificial Sequence: Synthetic polypeptide"
EVQLVESGGGLVKPGGSLRLSCAASGFTFNTYAMNWVRQAPGKGLEWVGRIRSKYNNYATYYADSVKDRFTISRDDSKNTLYLQMNSLKTEDTAVYYCTTHGNFGNSYVSWFAYWGQGTLVTVSSASTKGPSVFPLAPSSKSTSGGTAALGCLVKDYFPEPVTVSWNSGALTSGVHTFPAVLQSSGLYSLSSVVTVPSSSLGTQTYICNVNHKPSNTKVDKRVEPKSCDKTHTCPPCPAPEAEGAPSVFLFPPKPKDTLMISRTPEVTCVVVDVSHEDPEVKFNWYVDGVEVHNAKTKPREEQYNSTYRVVSVLTVLHQDWLNGKEYKCKVSNKALPSSIEKTISKAKGQPREPQVYTLPPSREEMTKNQVSLTCLVKGFYPSDIAVEWESNGQPENNYKTTPPVLDSDGSFFLYSKLTVDKSRWQQGNVFSCSVMHEALHNHYTQKSLSLSPGKASPAAPAPSADIQMTQSPSSLSASVGDRVTITCRASQDVNTAVAWYQQKPGKAPKLLIYSASFLYSGVPSRFSGSRSGTDFTLTISSLQPEDFATYYCQQHYTTPPTFGQGTKVEIKRTASPAAPAPASPAAPAPASGSQVQLVESGGGLVQPGGSLRLSCAASGFNIKDTYIHWVRQAPGKGLEWVARIYPTNGYTRYADSVKGRFTISADTSKNTAYLQMNSLRAEDTAVYYCSRWGGDGFYAMDYWGQGTLVTVSS

SEQ ID NO: 122 - DNA, 2142 bp, Artificial Sequence
  source: /note="Description of Artificial Sequence: Synthetic polynucleotide"
gaagtgcagctggtggaatctggcggcggactcgtgaagcctggcggctctctgagactgagctgtgccgccagcggcttcaccttcaacacctacgccatgaactgggtgcgccaggcccctggcaaaggcctggaatgggtgggacggatcagaagcaagtacaacaattacgccacctactacgccgacagcgtgaaggaccggttcaccatcagccgggacgacagcaagaacaccctgtacctgcagatgaacagcctgaaaaccgaggacaccgccgtgtactactgcaccacccacggcaacttcggcaacagctatgtgtcttggtttgcctactggggccagggcaccctcgtgacagtctcgagcgcgtcgaccaaaggccccagcgtgttccctctggcccccagcagcaagagcacctctggcggaacagccgccctgggctgcctggtcaaggactacttccccgagcccgtgaccgtgtcctggaactctggcgccctgaccagcggcgtgcacacctttccagccgtgctccagagcagcggcctgtacagcctgagcagcgtcgtgaccgtgcccagcagcagcctgggcacccagacctacatctgcaacgtgaaccacaagcccagcaacacaaaggtggacaagcgggtggaacccaagagctgcgacaagacccacacctgtcccccctgccctgcccctgaagcggagggagccccctccgtgttcctgttccccccaaagcctaaggacaccctgatgatcagccggacccccgaagtgacctgcgtggtggtggacgtgtcccacgaggaccctgaagtgaagtttaattggtacgtggacggcgtggaagtgcacaacgccaagaccaagcccagagaggaacagtacaacagcacctaccgggtggtgtccgtgctgaccgtgctgcaccaggactggctgaacggcaaagagtacaagtgcaaggtgtccaacaaggccctgccttcctccatcgagaaaaccatcagcaaggccaaaggccagccccgcgagccccaggtgtacacactgccccctagccgggaagagatgaccaagaaccaggtgtccctgacctgcctcgtgaagggcttctaccccagcgacattgccgtggaatgggagagcaacggccagcccgagaacaactacaagaccaccccccctgtgctggacagcgacggctcattcttcctgtacagcaagctgaccgtggacaagagccggtggcagcagggcaacgtgttcagctgctccgtgatgcacgaggccctgcacaaccactacacccagaagtccctgagcctgagccccggcaaggcttctcctgctgctcctgctcctagcgctgacatccagatgacccagagccctagcagcctgagcgccagcgtgggcgacagagtgaccatcacctgtagagccagccaggacgtgaacaccgccgtggcctggtatcagcagaagcctggcaaggcccccaagctgctgatctacagcgccagcttcctgtacagcggcgtgcccagcagattcagcggcagcagatccggcaccgacttcaccctgaccatcagcagcctgcagcccgaggacttcgccacctactactgccagcagcactacaccaccccccccacatttggccagggcaccaaggtggaaatcaagcggacagcctctcctgccgcccctgctcctgcttctcctgctgctccagctccagccagcggatctcaggtgcagctggtggaatctggcggcggactggtgcagcctggcggatctctgagactgagctgtgccgccagcggcttcaacatcaaggacacctacatccactgggtgcgccaggcccctggaaagggactggaatgggtggccagaatctaccccaccaacggctacaccagatacgccgacagcgtgaagggccggttcaccatcagcgccgacaccagcaagaataccgcctacctgcagatgaacagcctgagagccgaggataccgccgtgtactactgctccagatggggaggcgacggcttctacgccatggactattggggccagggaaccctcgtgaccgtgtcctct

SEQ ID NO: 123 - protein, 215 aa, Artificial Sequence; identical to SEQ ID NO: 71
  source: /note="Description of Artificial Sequence: Synthetic polypeptide"

SEQ ID NO: 124 - DNA, 645 bp, Artificial Sequence; identical to SEQ ID NO: 73
  source: /note="Description of Artificial Sequence: Synthetic polynucleotide"

SEQ ID NO: 125 - protein, 714 aa, Artificial Sequence; identical to SEQ ID NO: 121
  source: /note="Description of Artificial Sequence: Synthetic polypeptide"

SEQ ID NO: 126 - DNA, 2142 bp, Artificial Sequence; identical to SEQ ID NO: 122
  source: /note="Description of Artificial Sequence: Synthetic polynucleotide"

SEQ ID NO: 127 - protein, 215 aa, Artificial Sequence; identical to SEQ ID NO: 81
  source: /note="Description of Artificial Sequence: Synthetic polypeptide"

SEQ ID NO: 128 - DNA, 645 bp, Artificial Sequence; identical to SEQ ID NO: 83
  source: /note="Description of Artificial Sequence: Synthetic polynucleotide"

SEQ ID NO: 129 - protein, 714 aa, Artificial Sequence
  source: /note="Description of Artificial Sequence: Synthetic polypeptide"
QVQLVESGGGLVKPGGSLRLSCAASGFTFNTYAMNWIRQAPGKGLEWVSRIRSKYNNYATYYADSVKDRFTISRDNAKNSLYLQMNSLRAEDTAVYYCVRHGNFGNSYVSWFAYWGQGTLVTVSSASTKGPSVFPLAPSSKSTSGGTAALGCLVKDYFPEPVTVSWNSGALTSGVHTFPAVLQSSGLYSLSSVVTVPSSSLGTQTYICNVNHKPSNTKVDKRVEPKSCDKTHTCPPCPAPEAEGAPSVFLFPPKPKDTLMISRTPEVTCVVVDVSHEDPEVKFNWYVDGVEVHNAKTKPREEQYNSTYRVVSVLTVLHQDWLNGKEYKCKVSNKALPSSIEKTISKAKGQPREPQVYTLPPSREEMTKNQVSLTCLVKGFYPSDIAVEWESNGQPENNYKTTPPVLDSDGSFFLYSKLTVDKSRWQQGNVFSCSVMHEALHNHYTQKSLSLSPGKASPAAPAPSADIQMTQSPSSLSASVGDRVTITCRASQDVNTAVAWYQQKPGKAPKLLIYSASFLYSGVPSRFSGSRSGTDFTLTISSLQPEDFATYYCQQHYTTPPTFGQGTKVEIKRTASPAAPAPASPAAPAPASGSQVQLVESGGGLVQPGGSLRLSCAASGFNIKDTYIHWVRQAPGKGLEWVARIYPTNGYTRYADSVKGRFTISADTSKNTAYLQMNSLRAEDTAVYYCSRWGGDGFYAMDYWGQGTLVTVSS

SEQ ID NO: 130 - DNA, 2142 bp, Artificial Sequence
  source: /note="Description of Artificial Sequence: Synthetic polynucleotide"
caggtgcagctggtggaatctggcggcggactcgtgaagcctggcggctctctgagactgagctgtgccgccagcggcttcaccttcaacacctacgccatgaactggatccggcaggcccctggcaagggcctggaatgggtgtcccggatcagaagcaagtacaacaattacgccacctactacgccgacagcgtgaaggaccggttcaccatcagccgggacaacgccaagaacagcctgtacctgcagatgaactccctgcgggccgaggacaccgccgtgtactattgtgtgcggcacggcaacttcggcaacagctatgtgtcttggtttgcctactggggccagggcaccctcgtgacagtctcgagcgcgtcgaccaaaggccccagcgtgttccctctggcccccagcagcaagagcacctctggcggaacagccgccctgggctgcctggtcaaggactacttccccgagcccgtgaccgtgtcctggaactctggcgccctgaccagcggcgtgcacacctttccagccgtgctccagagcagcggcctgtacagcctgagcagcgtcgtgaccgtgcccagcagcagcctgggcacccagacctacatctgcaacgtgaaccacaagcccagcaacacaaaggtggacaagcgggtggaacccaagagctgcgacaagacccacacctgtcccccctgccctgcccctgaagcggagggagccccctccgtgttcctgttccccccaaagcctaaggacaccctgatgatcagccggacccccgaagtgacctgcgtggtggtggacgtgtcccacgaggaccctgaagtgaagtttaattggtacgtggacggcgtggaagtgcacaacgccaagaccaagcccagagaggaacagtacaacagcacctaccgggtggtgtccgtgctgaccgtgctgcaccaggactggctgaacggcaaagagtacaagtgcaaggtgtccaacaaggccctgccttcctccatcgagaaaaccatcagcaaggccaaaggccagccccgcgagccccaggtgtacacactgccccctagccgggaagagatgaccaagaaccaggtgtccctgacctgcctcgtgaagggcttctaccccagcgacattgccgtggaatgggagagcaacggccagcccgagaacaactacaagaccaccccccctgtgctggacagcgacggctcattcttcctgtacagcaagctgaccgtggacaagagccggtggcagcagggcaacgtgttcagctgctccgtgatgcacgaggccctgcacaaccactacacccagaagtccctgagcctgagccccggcaaggcttctcctgctgctcctgctcctagcgctgacatccagatgacccagagccctagcagcctgagcgccagcgtgggcgacagagtgaccatcacctgtagagccagccaggacgtgaacaccgccgtggcctggtatcagcagaagcctggcaaggcccccaagctgctgatctacagcgccagcttcctgtacagcggcgtgcccagcagattcagcggcagcagatccggcaccgacttcaccctgaccatcagcagcctgcagcccgaggacttcgccacctactactgccagcagcactacaccaccccccccacatttggccagggcaccaaggtggaaatcaagcggacagcctctcctgccgcccctgctcctgcttctcctgctgctccagctccagccagcggatctcaggtgcagctggtggaatctggcggcggactggtgcagcctggcggatctctgagactgagctgtgccgccagcggcttcaacatcaaggacacctacatccactgggtgcgccaggcccctggaaagggactggaatgggtggccagaatctaccccaccaacggctacaccagatacgccgacagcgtgaagggccggttcaccatcagcgccgacaccagcaagaataccgcctacctgcagatgaacagcctgagagccgaggataccgccgtgtactactgctccagatggggaggcgacggcttctacgccatggactattggggccagggaaccctcgtgaccgtgtcctct

SEQ ID NO: 131 - protein, 215 aa, Artificial Sequence; identical to SEQ ID NO: 39
  source: /note="Description of Artificial Sequence: Synthetic polypeptide"

SEQ ID NO: 132 - DNA, 645 bp, Artificial Sequence; identical to SEQ ID NO: 41
  source: /note="Description of Artificial Sequence: Synthetic polynucleotide"

SEQ ID NO: 133 - protein, 714 aa, Artificial Sequence; identical to SEQ ID NO: 129
  source: /note="Description of Artificial Sequence: Synthetic polypeptide"

SEQ ID NO: 134 - DNA, 2142 bp, Artificial Sequence; identical to SEQ ID NO: 130
  source: /note="Description of Artificial Sequence: Synthetic polynucleotide"

SEQ ID NO: 135 - protein, 215 aa, Artificial Sequence; identical to SEQ ID NO: 49
  source: /note="Description of Artificial Sequence: Synthetic polypeptide"

SEQ ID NO: 136 - DNA, 645 bp, Artificial Sequence; identical to SEQ ID NO: 51
  source: /note="Description of Artificial Sequence: Synthetic polynucleotide"

SEQ ID NO: 137 - protein, 714 aa, Artificial Sequence; identical to SEQ ID NO: 129
  source: /note="Description of Artificial Sequence: Synthetic polypeptide"

SEQ ID NO: 138 - DNA, 2142 bp, Artificial Sequence; identical to SEQ ID NO: 130
  source: /note="Description of Artificial Sequence: Synthetic polynucleotide"

SEQ ID NO: 139 - protein, 215 aa, Artificial Sequence; identical to SEQ ID NO: 81
  source: /note="Description of Artificial Sequence: Synthetic polypeptide"

SEQ ID NO: 140 - DNA, 645 bp, Artificial Sequence; identical to SEQ ID NO: 83
  source: /note="Description of Artificial Sequence: Synthetic polynucleotide"

SEQ ID NO: 141 - protein, 714 aa, Artificial Sequence; identical to SEQ ID NO: 129
  source: /note="Description of Artificial Sequence: Synthetic polypeptide"

SEQ ID NO: 142 - DNA, 2142 bp, Artificial Sequence; identical to SEQ ID NO: 130
  source: /note="Description of Artificial Sequence: Synthetic polynucleotide"

SEQ ID NO: 143 - protein, 215 aa, Artificial Sequence; identical to SEQ ID NO: 99
  source: /note="Description of Artificial Sequence: Synthetic polypeptide"

SEQ ID NO: 144 - DNA, 645 bp, Artificial Sequence; identical to SEQ ID NO: 101
  source: /note="Description of Artificial Sequence: Synthetic polynucleotide"

SEQ ID NO: 145 - protein, 714 aa, Artificial Sequence; identical to SEQ ID NO: 121
  source: /note="Description of Artificial Sequence: Synthetic polypeptide"

SEQ ID NO: 146 - DNA, 2142 bp, Artificial Sequence; identical to SEQ ID NO: 122
  source: /note="Description of Artificial Sequence: Synthetic polynucleotide"

SEQ ID NO: 147 - protein, 215 aa, Artificial Sequence; identical to SEQ ID NO: 59
  source: /note="Description of Artificial Sequence: Synthetic polypeptide"

SEQ ID NO: 148 - DNA, 645 bp, Artificial Sequence; identical to SEQ ID NO: 61
  source: /note="Description of Artificial Sequence: Synthetic polynucleotide"

SEQ ID NO: 149 - protein, 256 aa, Homo sapiens
QDGNEEMGGITQTPYKVSISGTTVILTCDIKTHTCPPCPAPELLGGPSVFLFPPKPKDTLMISRTPEVTCVVVDVSHEDPEVKFNWYVDGVEVHNAKTKPREEQYNSTYRVVSVLTVLHQDWLNGKEYKCKVSNKALPAPIEKTISKAKGQPREPQVYTLPPSREEMTKNQVSLTCLVKGFYPSDIAVEWESNGQPENNYKTTPPVLDSDGSFFLYSKLTVDKSRWQQGNVFSCSVMHEALHNHYTQKSLSLSPGK

SEQ ID NO: 150 - protein, 256 aa, Macaca fascicularis
QDGNEEMGSITQTPYQVSISGTTVILTCDIKTHTCPPCPAPELLGGPSVFLFPPKPKDTLMISRTPEVTCVVVDVSHEDPEVKFNWYVDGVEVHNAKTKPREEQYNSTYRVVSVLTVLHQDWLNGKEYKCKVSNKALPAPIEKTISKAKGQPREPQVYTLPPSREEMTKNQVSLTCLVKGFYPSDIAVEWESNGQPENNYKTTPPVLDSDGSFFLYSKLTVDKSRWQQGNVFSCSVMHEALHNHYTQKSLSLSPGK

SEQ ID NO: 151 - protein, 261 aa, Homo sapiens
QDGNEEMGGITQTPYKVSISGTTVILTCPQYPGSEILWQHNDKNIGGDEDDKNIGSDEDHLSLKEFSELEQSGYYVCYPRGSKPEDANFYLYLRARVDIDYKDDDDKIEGRMDKVFGRCELAAAMKRHGLDNYRGYSLGNWVCAAKFESNFNTQATNRNTDGSTDYGILQINSRWWCNDGRTPGSRNLCNIPCSALLSSDITASVNCAKKIVSDGNGMNAWVAWRNRCKGTDVQAWIRGCRLVNSRGLNDIFEAQKIEWHE

SEQ ID NO: 152 - protein, 120 aa, Artificial Sequence
  source: /note="Description of Artificial Sequence: Synthetic polypeptide"
QVQLVESGGGLVQPGGSLRLSCAASGFNIKDTYIHWVRQAPGKGLEWVARIYPTNGYTRYADSVKGRFTISADTSKNTAYLQMNSLRAEDTAVYYCSRWGGDGFYAMDYWGQGTLVTVSS

SEQ ID NO: 153 - protein, 109 aa, Artificial Sequence
  source: /note="Description of Artificial Sequence: Synthetic polypeptide"
DIQMTQSPSSLSASVGDRVTITCRASQDVNTAVAWYQQKPGKAPKLLIYSASFLYSGVPSRFSGSRSGTDFTLTISSLQPEDFATYYCQQHYTTPPTFGQGTKVEIKRT

SEQ ID NO: 154 - protein, 207 aa, Homo sapiens
MQSGTHWRVLGLCLLSVGVWGQDGNEEMGGITQTPYKVSISGTTVILTCPQYPGSEILWQHNDKNIGGDEDDKNIGSDEDHLSLKEFSELEQSGYYVCYPRGSKPEDANFYLYLRARVCENCMEMDVMSVATIVIVDICITGGLLLLVYYWSKNRKAKAKPVTRGAGAGGRQRGQNKERPPPVPNPDYEPIRKGQRDLYSGLNQRRI

SEQ ID NO: 155 - protein, 198 aa, Macaca fascicularis
MQSGTRWRVLGLCLLSIGVWGQDGNEEMGSITQTPYQVSISGTTVILTCSQHLGSEAQWQHNGKNKEDSGDRLFLPEFSEMEQSGYYVCYPRGSNPEDASHHLYLKARVCENCMEMDVMAVATIVIVDICITLGLLLLVYYWSKNRKAKAKPVTRGAGAGGRQRGQNKERPPPVPNPDYEPIRKGQQDLYSGLNQRRI

SEQ ID NO: 156 - protein, 266 aa, Artificial Sequence
  source: /note="Description of Artificial Sequence: Synthetic polypeptide"
ASPAAPAPSAQTVVTQEPSLTVSPGGTVTLTCRSSTGAVTTSNYANWVQQKPGQAPRGLIGGTKFLAPGTPARFSGSLLGGKAALTLSGVQPEDEAEYYCALWYSNLWVFGGGTKLTVLGQASPAAPAPASPAAPAPASGSEVQLVESGGGLVKPGGSLRLSCAASGFTFNTYAMNWVRQAPGKGLEWVGRIRSKYNNYATYYADSVKDRFTISRDDSKNTLYLQMNSLKTEDTAVYYCTTHGNFGNSYVSWFAYWGQGTLVTVSS

SEQ ID NO: 157 - DNA, 798 bp, Artificial Sequence
  source: /note="Description of Artificial Sequence: Synthetic polynucleotide"
gcttctcctgctgctcctgctcctagcgctcagaccgtggtcacacaagagcccagcctgacagtttctcctggcggcacagtgaccctgacctgcagatcttctacaggcgccgtgaccaccagcaactacgccaattgggtgcagcagaagcctggacaggctcccagaggactgatcggcggcacaaaatttctggcccctggcacaccagccagattctctggatctctgctcggcggaaaggccgctctgacactgtctggtgttcagcctgaggacgaggccgagtactattgcgccctgtggtacagcaacctgtgggtgttcggcggaggtaccaagctgaccgtgctgggccaggcctctcctgctgctcctgctccagcttctccagccgctccagctcctgctagcggatctgaagtgcagctggtggaatctggcggcggactcgtgaagcctggcggctctctgagactgagctgtgccgccagcggcttcaccttcaacacctacgccatgaactgggtgcgccaggcccctggcaaaggcctggaatgggtgggacggatcagaagcaagtacaacaattacgccacctactacgccgacagcgtgaaggaccggttcaccatcagccgggacgacagcaagaacaccctgtacctgcagatgaacagcctgaaaaccgaggacaccgccgtgtactactgcaccacccacggcaacttcggcaacagctatgtgtcttggtttgcctactggggccagggcaccctcgtgacagtctcgagc